European Patent Application EP 4 249 511 A2, published September 27, 2023. Title: ANTI-PD-L1/ANTI-LAG3 BISPECIFIC ANTIBODIES AND USES THEREOF. Applicant: ABL Bio Inc. Application EP. The sequence listing filed with the application follows.

SEQUENCE LISTING (555 sequences)

SEQ ID NO: 1 - protein, 5 aa, synthetic construct
  REGION 1..5: note = Synthetic
SYDMS

SEQ ID NO: 2 - protein, 17 aa, synthetic construct
  REGION 1..17: note = Synthetic
TISDGGGYIYYSDSVKG

SEQ ID NO: 3 - protein, 10 aa, synthetic construct
  REGION 1..10: note = Synthetic
EFGKRYALDY

SEQ ID NO: 4 - protein, 11 aa, synthetic construct
  REGION 1..11: note = Synthetic
KASQDVTPAVA

SEQ ID NO: 5 - protein, 7 aa, synthetic construct
  REGION 1..7: note = Synthetic
STSSRYT

SEQ ID NO: 6 - protein, 9 aa, synthetic construct
  REGION 1..9: note = Synthetic
QQHYTTPLT

SEQ ID NO: 7 - protein, 119 aa, synthetic construct
  REGION 1..119: note = Synthetic
EVKLVESGGDLVKPGGSLKLSCAASGFTFSSYDMSWVRQTPEKSLEWVATISDGGGYIYYSDSVKGRFTISRDNAKNNLYLQMSSLRSEDTALYICAREFGKRYALDYWGQGTSVTVSS

SEQ ID NO: 8 - protein, 119 aa, synthetic construct
  REGION 1..119: note = Synthetic
EVQLVESGGGLVKPGGSLRLSCAASGFTFSSYDMSWVRQAPGKGLEWVSTISDGGGYIYYSDSVKGRFTISRDNAKNSLYLQMNSLRAEDTAVYYCAREFGKRYALDYWGQGTTVTVSS

SEQ ID NO: 9 - protein, 119 aa, synthetic construct
  REGION 1..119: note = Synthetic
EVQLVESGGGLVKPGGSLRLSCAASGFTFSSYDMSWVRQAPGKGLEWVATISDGGGYIYYSDSVKGRFTISRDNAKNSLYLQMNSLRAEDTAVYYCAREFGKRYALDYWGQGTTVTVSS

SEQ ID NO: 10 - protein, 119 aa, synthetic construct
  REGION 1..119: note = Synthetic
EVQLVESGGGLVKPGGSLRLSCAASGFTFSSYDMSWVRQAPGKSLEWVATISDGGGYIYYSDSVKGRFTISRDNAKNSLYLQMNSLRAEDTAVYICAREFGKRYALDYWGQGTTVTVSS

SEQ ID NO: 11 - protein, 119 aa, synthetic construct
  REGION 1..119: note = Synthetic
EVQLVESGGGLVKPGGSLRLSCAASGFTFSSYDMSWIRQAPGKGLEWVSTISDGGGYIYYSDSVKGRFTISRDNAKNSLYLQMNSLRAEDTAVYYCAREFGKRYALDYWGQGTTVTVSS

SEQ ID NO: 12 - protein, 119 aa, synthetic construct
  REGION 1..119: note = Synthetic
EVQLVESGGGLVKPGGSLRLSCAASGFTFSSYDMSWIRQAPGKGLEWVATISDGGGYIYYSDSVKGRFTISRDNAKNSLYLQMNSLRAEDTAVYYCAREFGKRYALDYWGQGTTVTVSS

SEQ ID NO: 13 - protein, 119 aa, synthetic construct; identical to SEQ ID NO: 10
  REGION 1..119: note = Synthetic

SEQ ID NO: 14 - protein, 119 aa, synthetic construct
  REGION 1..119: note = Synthetic
EVQLLESGGGLVQPGGSLRLSCAASGFTFSSYDMSWVRQAPGKGLEWVSTISDGGGYIYYSDSVKGRFTISRDNSKNTLYLQMNSLRAEDTAVYYCAREFGKRYALDYWGQGTTVTVSS

SEQ ID NO: 15 - protein, 119 aa, synthetic construct
  REGION 1..119: note = Synthetic
EVQLLESGGGLVQPGGSLRLSCAASGFTFSSYDMSWVRQAPGKSLEWVATISDGGGYIYYSDSVKGRFTISRDNSKNTLYLQMNSLRAEDTAVYICAREFGKRYALDYWGQGTTVTVSS

SEQ ID NO: 16 - protein, 119 aa, synthetic construct
  REGION 1..119: note = Synthetic
EVQLVESGGGLVQPGGSLRLSCAASGFTFSSYDMSWVRQAPGKGLEWVSTISDGGGYIYYSDSVKGRFTISRDNAKNSLYLQMNSLRDEDTAVYYCAREFGKRYALDYWGQGTTVTVSS

SEQ ID NO: 17 - protein, 119 aa, synthetic construct
  REGION 1..119: note = Synthetic
EVQLVESGGGLVQPGGSLRLSCAASGFTFSSYDMSWVRQAPGKGLEWVATISDGGGYIYYSDSVKGRFTISRDNAKNSLYLQMNSLRDEDTAVYYCAREFGKRYALDYWGQGTTVTVSS

SEQ ID NO: 18 - protein, 119 aa, synthetic construct
  REGION 1..119: note = Synthetic
EVQLVESGGGLVQPGGSLRLSCAASGFTFSSYDMSWVRQAPGKSLEWVATISDGGGYIYYSDSVKGRFTISRDNAKNSLYLQMNSLRDEDTAVYICAREFGKRYALDYWGQGTTVTVSS

SEQ ID NO: 19 - protein, 119 aa, synthetic construct
  REGION 1..119: note = Synthetic
EVQLVESGGGLVQPGGSLRLSCAASGFTFSSYDMSWVRQAPGKSLEWVATISEGGGYIYYSDSVKGRFTISRDNAKNSLYLQMNSLRDEDTAVYICAREFGKRYALDYWGQGTTVTVSS

SEQ ID NO: 20 - protein, 119 aa, synthetic construct
  REGION 1..119: note = Synthetic
EVQLVESGGGLVQPGGSLRLSCAASGFTFSSYDMSWVRQAPGKSLEWVATISDAGGYIYYSDSVKGRFTISRDNAKNSLYLQMNSLRDEDTAVYICAREFGKRYALDYWGQGTTVTVSS

SEQ ID NO: 21 - protein, 119 aa, synthetic construct
  REGION 1..119: note = Synthetic
EVQLVESGGGLVQPGGSLRLSCAASGFTFSSYDMSWVRQAPGKSLEWVATISDVGGYIYYSDSVKGRFTISRDNAKNSLYLQMNSLRDEDTAVYICAREFGKRYALDYWGQGTTVTVSS

SEQ ID NO: 22 - protein, 119 aa, synthetic construct
  REGION 1..119: note = Synthetic
EVQLVESGGGLVQPGGSLRLSCAASGFTFSSYDMSWVRQAPGKGLEWVATISDGGGYIYYSDSVKGRFTISRDNAKNSLYLQMNSLRAEDTAVYYCAREFGKRYALDYWGQGTLVTVSS

SEQ ID NO: 23 - protein, 119 aa, synthetic construct
  REGION 1..119: note = Synthetic
EVQLVESGGGLVQPGGSLRLSCAASGFTFSSYDMSWVRQAPGKGLEWVATISDGGGYIYYSDSVKGRFTISRDNAKNSLYLQMNSLRAEDTAVYICAREFGKRYALDYWGQGTLVTVSS

SEQ ID NO: 24 - protein, 119 aa, synthetic construct
  REGION 1..119: note = Synthetic
EVQLVESGGGLVQPGGSLRLSCAASGFTFSSYDMSWVRQAPGKGLEWVATISDGGGYIYYSDSVKGRFTISRDNAKNSLYLQMNSLRAEDTAVYICAREFGKRYALDYWGQGTTVTVSS

SEQ ID NO: 25 - protein, 119 aa, synthetic construct
  REGION 1..119: note = Synthetic
EVQLVESGGGLVQPGGSLRLSCAASGFTFSSYDMSWVRQAPGKGLEWVATISDGGGYIYYSDSVKGRFTISRDNAKNNLYLQMNSLRAEDTAVYICAREFGKRYALDYWGQGTLVTVSS

SEQ ID NO: 26 - protein, 119 aa, synthetic construct
  REGION 1..119: note = Synthetic
EVQLVESGGGLVQPGGSLRLSCAASGFTFSSYDMSWVRQTPEKSLEWVATISDGGGYIYYSDSVKGRFTISRDNAKNNLYLQMNSLRAEDTAVYICAREFGKRYALDYWGQGTLVTVSS

SEQ ID NO: 27 - protein, 107 aa, synthetic construct
  REGION 1..107: note = Synthetic
DIVMTQSHKFMSTSVGDRVSISCKASQDVTPAVAWYQQKPGQSPKLLIYSTSSRYTGVPDRFTGSGSGTDFTFTISSVQAEDLAVYYCQQHYTTPLTFGAGTKLELK

SEQ ID NO: 28 - protein, 107 aa, synthetic construct
  REGION 1..107: note = Synthetic
DIQMTQSPSSLSASVGDRVTITCKASQDVTPAVAWYQQKPGKAPKLLIYSTSSRYTGVPSRFSGSGSGTDFTFTISSLQPEDIATYYCQQHYTTPLTFGQGTKLEIK

SEQ ID NO: 29 - protein, 107 aa, synthetic construct
  REGION 1..107: note = Synthetic
DIQMTQSPSSLSASVGDRVTITCKASQDVTPAVAWYQQKPGKSPKLLIYSTSSRYTGVPSRFSGSGSGTDFTFTISSLQPEDIATYYCQQHYTTPLTFGQGTKLEIK

SEQ ID NO: 30 - protein, 108 aa, synthetic construct
  REGION 1..108: note = Synthetic
DIQMTQSPSSLSASVGDRVTITCKASQDVTPAVAWYQQKPGKAPKLLIYSTSSRYTGVPSRFSGSGSGTDFTLTISSLQPEDFATYYCQQHYTTPLTFGQGTKLEIKR

SEQ ID NO: 31 - protein, 108 aa, synthetic construct
  REGION 1..108: note = Synthetic
DIQMTQSPSSLSASVGDRVTITCKASQDVTPAVAWYQQKPGKAPKLLIYSTSSRYTGVPDRFTGSGSGTDFTLTISSLQPEDFATYYCQQHYTTPLTFGQGTKLEIKR

SEQ ID NO: 32 - protein, 108 aa, synthetic construct
  REGION 1..108: note = Synthetic
DIQMTQSPSSLSASVGDRVTITCKASQDVTPAVAWYQQKPGQSPKLLIYSTSSRYTGVPDRFTGSGSGTDFTLTISSLQPEDFATYYCQQHYTTPLTFGQGTKLEIKR

SEQ ID NO: 33 - protein, 108 aa, synthetic construct
  REGION 1..108: note = Synthetic
DIQMTQSPSSLSASVGDRVTISCKASQDVTPAVAWYQQKPGQSPKLLIYSTSSRYTGVPDRFTGSGSGTDFTLTISSLQPEDFATYYCQQHYTTPLTFGQGTKLEIKR

SEQ ID NO: 34 - DNA, 357 bp, synthetic construct
  misc_feature 1..357: note = Synthetic
  source 1..357: mol_type = other DNA
gaggtgaagctggtggagagcggcggagatctggtgaagcctggcggcagcctgaagctgagctgtgccgccagcggcttcaccttcagcagctacgacatgagctgggtgaggcagacccccgagaagagcctggagtgggtggccaccatcagcgatggcggcggctacatctactacagcgacagcgtgaagggcaggttcaccatcagcagggacaacgccaagaacaacctgtacctgcagatgagcagcctgaggagcgaggacaccgccctgtacatctgcgccagggagttcggcaagaggtacgccctggactactggggacagggcaccagcgtgaccgtgagcagc

SEQ ID NO: 35 - DNA, 357 bp, synthetic construct
  misc_feature 1..357: note = Synthetic
  source 1..357: mol_type = other DNA
gaggtgcagctggtggagagcggaggaggactggtgaagcccggaggcagcctgagactgagctgcgctgccagcggcttcaccttcagcagctacgacatgagctgggtgagacaggcccctggcaaaggcctggagtgggtgagcaccatctccgatggcggcggctacatctattactccgacagcgtgaagggcaggttcaccatcagcagggacaacgccaagaacagcctgtacctgcagatgaacagcctgagggccgaggacaccgccgtgtactactgcgccagggagttcggcaaaaggtacgccctggactactggggccagggcacaaccgtgaccgtgagcagc

SEQ ID NO: 36 - DNA, 357 bp, synthetic construct
  misc_feature 1..357: note = Synthetic
  source 1..357: mol_type = other DNA
gaggtgcagctggtggagagcggaggaggactggtgaagcccggaggcagcctgagactgagctgcgctgccagcggcttcaccttcagcagctacgacatgagctgggtgagacaggcccctggcaaaggcctggagtgggtggccaccatctccgatggcggcggctacatctattactccgacagcgtgaagggcaggttcaccatcagcagggacaacgccaagaacagcctgtacctgcagatgaacagcctgagggccgaggacaccgccgtgtactactgcgccagggagttcggcaaaaggtacgccctggactactggggccagggcacaaccgtgaccgtgagcagc

SEQ ID NO: 37 - DNA, 357 bp, synthetic construct
  misc_feature 1..357: note = Synthetic
  source 1..357: mol_type = other DNA
gaggtgcagctggtggagagcggaggaggactggtgaagcccggaggcagcctgagactgagctgcgctgccagcggcttcaccttcagcagctacgacatgagctgggtgagacaggcccctggcaaaagcctggagtgggtggccaccatctccgatggcggcggctacatctattactccgacagcgtgaagggcaggttcaccatcagcagggacaacgccaagaacagcctgtacctgcagatgaacagcctgagggccgaggacaccgccgtgtacatctgcgccagggagttcggcaaaaggtacgccctggactactggggccagggcacaaccgtgaccgtgagcagc

SEQ ID NO: 38 - DNA, 357 bp, synthetic construct
  misc_feature 1..357: note = Synthetic
  source 1..357: mol_type = other DNA
gaggtgcagctggtggagagcggaggaggactggtgaagcccggaggcagcctgagactgagctgcgctgccagcggcttcaccttcagcagctacgacatgagctggatcagacaggcccctggcaaaggcctggagtgggtgagcaccatctccgatggcggcggctacatctattactccgacagcgtgaagggcaggttcaccatcagcagggacaacgccaagaacagcctgtacctgcagatgaacagcctgagggccgaggacaccgccgtgtactactgcgccagggagttcggcaaaaggtacgccctggactactggggccagggcacaaccgtgaccgtgagcagc

SEQ ID NO: 39 - DNA, 357 bp, synthetic construct
  misc_feature 1..357: note = Synthetic
  source 1..357: mol_type = other DNA
gaggtgcagctggtggagagcggaggaggactggtgaagcccggaggcagcctgagactgagctgcgctgccagcggcttcaccttcagcagctacgacatgagctggatcagacaggcccctggcaaaggcctggagtgggtggccaccatctccgatggcggcggctacatctattactccgacagcgtgaagggcaggttcaccatcagcagggacaacgccaagaacagcctgtacctgcagatgaacagcctgagggccgaggacaccgccgtgtactactgcgccagggagttcggcaaaaggtacgccctggactactggggccagggcacaaccgtgaccgtgagcagc

SEQ ID NO: 40 - DNA, 357 bp, synthetic construct; identical to SEQ ID NO: 37
  misc_feature 1..357: note = Synthetic
  source 1..357: mol_type = other DNA

SEQ ID NO: 41 - DNA, 357 bp, synthetic construct
  misc_feature 1..357: note = Synthetic
  source 1..357: mol_type = other DNA
gaggtgcagctgctggagagcggaggaggactggtgcaacccggaggcagcctgagactgagctgcgctgccagcggcttcaccttcagcagctacgacatgagctgggtgagacaggcccctggcaaaggcctggagtgggtgagcaccatctccgatggcggcggctacatctattactccgacagcgtgaagggcaggttcaccatcagcagggacaacagcaagaacaccctgtacctgcagatgaacagcctgagggccgaggacaccgccgtgtactactgcgccagggagttcggcaaaaggtacgccctggactactggggccagggcacaaccgtgaccgtgagcagc

SEQ ID NO: 42 - DNA, 357 bp, synthetic construct
  misc_feature 1..357: note = Synthetic
  source 1..357: mol_type = other DNA
gaggtgcagctgctggagagcggaggaggactggtgcaacccggaggcagcctgagactgagctgcgctgccagcggcttcaccttcagcagctacgacatgagctgggtgagacaggcccctggcaaaagcctggagtgggtggccaccatctccgatggcggcggctacatctattactccgacagcgtgaagggcaggttcaccatcagcagggacaacagcaagaacaccctgtacctgcagatgaacagcctgagggccgaggacaccgccgtgtacatctgcgccagggagttcggcaaaaggtacgccctggactactggggccagggcacaaccgtgaccgtgagcagc

SEQ ID NO: 43 - DNA, 357 bp, synthetic construct
  misc_feature 1..357: note = Synthetic
  source 1..357: mol_type = other DNA
gaggtgcagctggtggagagcggaggaggactggtgcaacccggaggcagcctgagactgagctgcgctgccagcggcttcaccttcagcagctacgacatgagctgggtgagacaggcccctggcaaaggcctggagtgggtgagcaccatctccgatggcggcggctacatctattactccgacagcgtgaagggcaggttcaccatcagcagggacaacgccaagaacagcctgtacctgcagatgaacagcctgagggatgaggacaccgccgtgtactactgcgccagggagttcggcaaaaggtacgccctggactactggggccagggcacaaccgtgaccgtgagcagc

SEQ ID NO: 44 - DNA, 357 bp, synthetic construct
  misc_feature 1..357: note = Synthetic
  source 1..357: mol_type = other DNA
gaggtgcagctggtggagagcggaggaggactggtgcaacccggaggcagcctgagactgagctgcgctgccagcggcttcaccttcagcagctacgacatgagctgggtgagacaggcccctggcaaaggcctggagtgggtggccaccatctccgatggcggcggctacatctattactccgacagcgtgaagggcaggttcaccatcagcagggacaacgccaagaacagcctgtacctgcagatgaacagcctgagggatgaggacaccgccgtgtactactgcgccagggagttcggcaaaaggtacgccctggactactggggccagggcacaaccgtgaccgtgagcagc

SEQ ID NO: 45 - DNA, 357 bp, synthetic construct
  misc_feature 1..357: note = Synthetic
  source 1..357: mol_type = other DNA
gaggtgcagctggtggagagcggaggaggactggtgcaacccggaggcagcctgagactgagctgcgctgccagcggcttcaccttcagcagctacgacatgagctgggtgagacaggcccctggcaaaagcctggagtgggtggccaccatctccgatggcggcggctacatctattactccgacagcgtgaagggcaggttcaccatcagcagggacaacgccaagaacagcctgtacctgcagatgaacagcctgagggatgaggacaccgccgtgtacatctgcgccagggagttcggcaaaaggtacgccctggactactggggccagggcacaaccgtgaccgtgagcagc

SEQ ID NO: 46 - DNA, 357 bp, synthetic construct
  misc_feature 1..357: note = Synthetic
  source 1..357: mol_type = other DNA
gaggtgcagctggtggagagcggaggaggactggtgcaacccggaggcagcctgagactgagctgcgctgccagcggcttcaccttcagcagctacgacatgagctgggtgagacaggcccctggcaaaagcctggagtgggtggccaccatctccgaaggcggcggctacatctattactccgacagcgtgaagggcaggttcaccatcagcagggacaacgccaagaacagcctgtacctgcagatgaacagcctgagggatgaggacaccgccgtgtacatctgcgccagggagttcggcaaaaggtacgccctggactactggggccagggcacaaccgtgaccgtgagcagc

SEQ ID NO: 47 - DNA, 357 bp, synthetic construct
  misc_feature 1..357: note = Synthetic
  source 1..357: mol_type = other DNA
gaggtgcagctggtggagagcggaggaggactggtgcaacccggaggcagcctgagactgagctgcgctgccagcggcttcaccttcagcagctacgacatgagctgggtgagacaggcccctggcaaaagcctggagtgggtggccaccatctccgatgcgggcggctacatctattactccgacagcgtgaagggcaggttcaccatcagcagggacaacgccaagaacagcctgtacctgcagatgaacagcctgagggatgaggacaccgccgtgtacatctgcgccagggagttcggcaaaaggtacgccctggactactggggccagggcacaaccgtgaccgtgagcagc

SEQ ID NO: 48 - DNA, 357 bp, synthetic construct
  misc_feature 1..357: note = Synthetic
  source 1..357: mol_type = other DNA
gaggtgcagctggtggagagcggaggaggactggtgcaacccggaggcagcctgagactgagctgcgctgccagcggcttcaccttcagcagctacgacatgagctgggtgagacaggcccctggcaaaagcctggagtgggtggccaccatctccgatgttggcggctacatctattactccgacagcgtgaagggcaggttcaccatcagcagggacaacgccaagaacagcctgtacctgcagatgaacagcctgagggatgaggacaccgccgtgtacatctgcgccagggagttcggcaaaaggtacgccctggactactggggccagggcacaaccgtgaccgtgagcagc

SEQ ID NO: 49 - DNA, 357 bp, synthetic construct
  misc_feature 1..357: note = Synthetic
  source 1..357: mol_type = other DNA
gaggtgcagctggtggagtccggaggaggcctggtgcaacctggaggctccctgaggctgtcctgtgccgcttccggcttcaccttcagctcctacgatatgagctgggtgaggcaggctcctggaaagggcctggagtgggtggccaccatctccgacggaggcggctacatctactactccgactccgtgaagggcaggttcaccatctcccgggacaacgccaagaactccctgtacctgcagatgaactctctcagggctgaggacaccgccgtgtattactgcgccagggagtttggcaagaggtacgccctggattactggggccagggcacactggtgacagtgagctcc

SEQ ID NO: 50 - DNA, 357 bp, synthetic construct
  misc_feature 1..357: note = Synthetic
  source 1..357: mol_type = other DNA
gaggtgcagctggtggagtccggaggaggcctggtgcaacctggaggctccctgaggctgtcctgtgccgcttccggcttcaccttcagctcctacgatatgagctgggtgaggcaggctcctggaaagggcctggagtgggtggccaccatctccgacggaggcggctacatctactactccgactccgtgaagggcaggttcaccatctcccgggacaacgccaagaactccctgtacctgcagatgaactctctcagggctgaggacaccgccgtgtatatctgcgccagggagtttggcaagaggtacgccctggattactggggccagggcacactggtgacagtgagctcc

SEQ ID NO: 51 - DNA, 357 bp, synthetic construct
  misc_feature 1..357: note = Synthetic
  source 1..357: mol_type = other DNA
gaggtgcagctggtggagtccggaggaggcctggtgcaacctggaggctccctgaggctgtcctgtgccgcttccggcttcaccttcagctcctacgatatgagctgggtgaggcaggctcctggaaagggcctggagtgggtggccaccatctccgacggaggcggctacatctactactccgactccgtgaagggcaggttcaccatctcccgggacaacgccaagaacaacctgtacctgcagatgaactctctcagggctgaggacaccgccgtgtatatctgcgccagggagtttggcaagaggtacgccctggattactggggccagggcacactggtgacagtgagctcc

SEQ ID NO: 52 - DNA, 357 bp, synthetic construct
  misc_feature 1..357: note = Synthetic
  source 1..357: mol_type = other DNA
gaggtgcagctggtggagtccggaggaggcctggtgcaacctggaggctccctgaggctgtcctgtgccgcttccggcttcaccttcagctcctacgatatgagctgggtgaggcagacccctgagaagagcctggagtgggtggccaccatctccgacggaggcggctacatctactactccgactccgtgaagggcaggttcaccatctcccgggacaacgccaagaacaacctgtacctgcagatgaactctctcagggctgaggacaccgccgtgtatatctgcgccagggagtttggcaagaggtacgccctggattactggggccagggcacactggtgacagtgagctcc

SEQ ID NO: 53 - DNA, 357 bp, synthetic construct
  misc_feature 1..357: note = Synthetic
  source 1..357: mol_type = other DNA
gaggtgcagctggtggagtccggaggaggcctggtgcaacctggaggctccctgaggctgtcctgtgccgcttccggcttcaccttcagctcctacgatatgagctgggtgaggcaggctcctggaaagggcctggagtgggtggccaccatctccgacggaggcggctacatctactactccgactccgtgaagggcaggttcaccatctcccgggacaacgccaagaactccctgtacctgcagatgaactctctcagggctgaggacaccgccgtgtatatctgcgccagggagtttggcaagaggtacgccctggattactggggccagggcacaaccgtgacagtgagctcc

SEQ ID NO: 54 - DNA, 321 bp, synthetic construct
  misc_feature 1..321: note = Synthetic
  source 1..321: mol_type = other DNA
gacatcgtgatgacccagagccacaagttcatgagcaccagcgtgggcgatagggtgagcatcagctgcaaggccagccaggatgtgacccctgccgtggcctggtaccagcagaagcccggccagagccccaagctgctgatctacagcaccagcagcaggtacaccggcgtgcccgacaggttcacaggaagcggcagcggcaccgacttcaccttcaccatcagcagcgtgcaggccgaggacctggccgtgtactactgccagcagcactacaccacccctctgaccttcggcgccggcaccaagctggagctgaag

SEQ ID NO: 55 - DNA, 321 bp, synthetic construct
  misc_feature 1..321: note = Synthetic
  source 1..321: mol_type = other DNA
gacatccagatgacccagagccctagcagcctgagcgctagcgtgggcgacagggtgaccatcacctgcaaggccagccaggatgtgacccctgccgtggcctggtaccagcagaagcccggcaaggcccccaagctgctgatctacagcaccagcagcaggtacaccggcgtgcccagcaggtttagcggaagcggcagcggcaccgacttcaccttcaccatcagcagcctgcagcccgaggacatcgccacctactactgccagcagcactacaccacccctctgaccttcggccagggcaccaagctggagatcaag

SEQ ID NO: 56 - DNA, 321 bp, synthetic construct
  misc_feature 1..321: note = Synthetic
  source 1..321: mol_type = other DNA
gacatccagatgacccagagccctagcagcctgagcgctagcgtgggcgacagggtgaccatcacctgcaaggccagccaggatgtgacccctgccgtggcctggtaccagcagaagcccggcaagtcccccaagctgctgatctacagcaccagcagcaggtacaccggcgtgcccagcaggtttagcggaagcggcagcggcaccgacttcaccttcaccatcagcagcctgcagcccgaggacatcgccacctactactgccagcagcactacaccacccctctgaccttcggccagggcaccaagctggagatcaag

SEQ ID NO: 57 - DNA, 324 bp, synthetic construct
  misc_feature 1..324: note = Synthetic
  source 1..324: mol_type = other DNA
gacattcagatgacccagtcccctagcagcctgtccgcttccgtgggcgacagggtgaccatcacctgcaaggccagccaggacgtgacacctgctgtggcctggtatcaacagaagcctggcaaggctcctaagctcctgatctacagcacatcctcccggtacaccggagtgccctccaggtttagcggcagcggctccggcaccgatttcaccctgaccatttcctccctgcagcccgaggacttcgccacctactactgccagcagcactacaccacacccctgaccttcggccagggcaccaagctggagatcaagcgg

SEQ ID NO: 58 - DNA, 324 bp, synthetic construct
  misc_feature 1..324: note = Synthetic
  source 1..324: mol_type = other DNA
gacattcagatgacccagtcccctagcagcctgtccgcttccgtgggcgacagggtgaccatcacctgcaaggccagccaggacgtgacacctgctgtggcctggtatcaacagaagcctggcaaggctcctaagctcctgatctacagcacatcctcccggtacaccggagtgcccgacaggtttaccggcagcggctccggcaccgatttcaccctgaccatttcctccctgcagcccgaggacttcgccacctactactgccagcagcactacaccacacccctgaccttcggccagggcaccaagctggagatcaagcgg

SEQ ID NO: 59 - DNA, 324 bp, synthetic construct
  misc_feature 1..324: note = Synthetic
  source 1..324: mol_type = other DNA
gacattcagatgacccagtcccctagcagcctgtccgcttccgtgggcgacagggtgaccatcacctgcaaggccagccaggacgtgacacctgctgtggcctggtatcaacagaagcctggccagagccctaagctcctgatctacagcacatcctcccggtacaccggagtgcccgacaggtttaccggcagcggctccggcaccgatttcaccctgaccatttcctccctgcagcccgaggacttcgccacctactactgccagcagcactacaccacacccctgaccttcggccagggcaccaagctggagatcaagcgg

SEQ ID NO: 60 - DNA, 324 bp, synthetic construct
  misc_feature 1..324: note = Synthetic
  source 1..324: mol_type = other DNA
gacattcagatgacccagtcccctagcagcctgtccgcttccgtgggcgacagggtgaccatcagctgcaaggccagccaggacgtgacacctgctgtggcctggtatcaacagaagcctggccagagccctaagctcctgatctacagcacatcctcccggtacaccggagtgcccgacaggtttaccggcagcggctccggcaccgatttcaccctgaccatttcctccctgcagcccgaggacttcgccacctactactgccagcagcactacaccacacccctgaccttcggccagggcaccaagctggagatcaagcgg

SEQ ID NO: 61 - protein, 5 aa, synthetic construct
  REGION 1..5: note = Synthetic
TYDMS

SEQ ID NO: 62 - protein, 5 aa, synthetic construct
  REGION 1..5: note = Synthetic
CYDMS

SEQ ID NO: 63 - protein, 5 aa, synthetic construct
  REGION 1..5: note = Synthetic
SFDMS

SEQ ID NO: 64 - protein, 5 aa, synthetic construct
  REGION 1..5: note = Synthetic
SHDMS

SEQ ID NO: 65 - protein, 5 aa, synthetic construct
  REGION 1..5: note = Synthetic
SWDMS

SEQ ID NO: 66 - protein, 5 aa, synthetic construct
  REGION 1..5: note = Synthetic
SYDMT

SEQ ID NO: 67 - protein, 5 aa, synthetic construct
  REGION 1..5: note = Synthetic
SYDMC

SEQ ID NO: 68 - protein, 17 aa, synthetic construct
  REGION 1..17: note = Synthetic
TISDGGAYIYYSDSVKG

SEQ ID NO: 69 - protein, 17 aa, synthetic construct
  REGION 1..17: note = Synthetic
TISDGGPYIYYSDSVKG

SEQ ID NO: 70 - protein, 17 aa, synthetic construct
  REGION 1..17: note = Synthetic
TISDGGGFIYYSDSVKG

SEQ ID NO: 71 - protein, 17 aa, synthetic construct
  REGION 1..17: note = Synthetic
TISDGGGHIYYSDSVKG

SEQ ID NO: 72 - protein, 17 aa, synthetic construct
  REGION 1..17: note = Synthetic
TISDGGGWIYYSDSVKG

SEQ ID NO: 73 - protein, 17 aa, synthetic construct
  REGION 1..17: note = Synthetic
TISDGGGYIYYSDTVKG

SEQ ID NO: 74 - protein, 17 aa, synthetic construct
  REGION 1..17: note = Synthetic
TISDGGGYIYYSDCVKG

SEQ ID NO: 75 - protein, 17 aa, synthetic construct
  REGION 1..17: note = Synthetic
TISDGGGYIYYSDSLKG

SEQ ID NO: 76 - protein, 17 aa, synthetic construct
  REGION 1..17: note = Synthetic
TISDGGGYIYYSDSIKG

SEQ ID NO: 77 - protein, 17 aa, synthetic construct
  REGION 1..17: note = Synthetic
TISDGGGYIYYSDSMKG

SEQ ID NO: 78 - protein, 10 aa, synthetic construct
  REGION 1..10: note = Synthetic
QFGKRYALDY

SEQ ID NO: 79 - protein, 10 aa, synthetic construct
  REGION 1..10: note = Synthetic
DFGKRYALDY

SEQ ID NO: 80 - protein, 10 aa, synthetic construct
  REGION 1..10: note = Synthetic
NFGKRYALDY

SEQ ID NO: 81 - protein, 10 aa, synthetic construct
  REGION 1..10: note = Synthetic
EYGKRYALDY

SEQ ID NO: 82 - protein, 10 aa, synthetic construct
  REGION 1..10: note = Synthetic
EHGKRYALDY

SEQ ID NO: 83 - protein, 10 aa, synthetic construct
  REGION 1..10: note = Synthetic
EWGKRYALDY

SEQ ID NO: 84 - protein, 10 aa, synthetic construct
  REGION 1..10: note = Synthetic
EFAKRYALDY

SEQ ID NO: 85 - protein, 10 aa, synthetic construct
  REGION 1..10: note = Synthetic
EFPKRYALDY

SEQ ID NO: 86 - protein, 10 aa, synthetic construct
  REGION 1..10: note = Synthetic
EFGRRYALDY

SEQ ID NO: 87 - protein, 10 aa, synthetic construct
  REGION 1..10: note = Synthetic
EFGKKYALDY

SEQ ID NO: 88 - protein, 10 aa, synthetic construct
  REGION 1..10: note = Synthetic
EFGKRFALDY

SEQ ID NO: 89 - protein, 10 aa, synthetic construct
  REGION 1..10: note = Synthetic
EFGKRHALDY

SEQ ID NO: 90 - protein, 10 aa, synthetic construct
  REGION 1..10: note = Synthetic
EFGKRWALDY

SEQ ID NO: 91 - protein, 11 aa, synthetic construct
  REGION 1..11: note = Synthetic
KATQDVTPAVA

SEQ ID NO: 92 - protein, 11 aa, synthetic construct
  REGION 1..11: note = Synthetic
KACQDVTPAVA

SEQ ID NO: 93 - protein, 7 aa, synthetic construct
  REGION 1..7: note = Synthetic
TTSSRYT

SEQ ID NO: 94 - protein, 7 aa, synthetic construct
  REGION 1..7: note = Synthetic
CTSSRYT

SEQ ID NO: 95 - protein, 7 aa, synthetic construct
  REGION 1..7: note = Synthetic
SSSSRYT

SEQ ID NO: 96 - protein, 7 aa, synthetic construct
  REGION 1..7: note = Synthetic
SMSSRYT

SEQ ID NO: 97 - protein, 7 aa, synthetic construct
  REGION 1..7: note = Synthetic
SVSSRYT

SEQ ID NO: 98 - protein, 7 aa, synthetic construct
  REGION 1..7: note = Synthetic
STTSRYT

SEQ ID NO: 99 - protein, 7 aa, synthetic construct
  REGION 1..7: note = Synthetic
STCSRYT

SEQ ID NO: 100 - protein, 7 aa, synthetic construct
  REGION 1..7: note = Synthetic
STSTRYT

SEQ ID NO: 101 - protein, 7 aa, synthetic construct
  REGION 1..7: note = Synthetic
STSCRYT

SEQ ID NO: 102 - protein, 7 aa, synthetic construct
  REGION 1..7: note = Synthetic
STSSKYT

SEQ ID NO: 103 - protein, 7 aa, synthetic construct
  REGION 1..7: note = Synthetic
STSSRFT

SEQ ID NO: 104 - protein, 7 aa, synthetic construct
  REGION 1..7: note = Synthetic
STSSRHT

SEQ ID NO: 105 - protein, 7 aa, synthetic construct
  REGION 1..7: note = Synthetic
STSSRWT

SEQ ID NO: 106 - protein, 9 aa, synthetic construct
  REGION 1..9: note = Synthetic
EQHYTTPLT

SEQ ID NO: 107 - protein, 9 aa, synthetic construct
  REGION 1..9: note = Synthetic
DQHYTTPLT

SEQ ID NO: 108 - protein, 9 aa, synthetic construct
  REGION 1..9: note = Synthetic
NQHYTTPLT

SEQ ID NO: 109 - protein, 9 aa, synthetic construct
  REGION 1..9: note = Synthetic
QEHYTTPLT

SEQ ID NO: 110 - protein, 9 aa, synthetic construct
  REGION 1..9: note = Synthetic
QDHYTTPLT

SEQ ID NO: 111 - protein, 9 aa, synthetic construct
  REGION 1..9: note = Synthetic
QNHYTTPLT

SEQ ID NO: 112 - DNA, 357 bp, synthetic construct
  misc_feature 1..357: note = Synthetic
  source 1..357: mol_type = other DNA
gaagtgaaactggtggagtctgggggagacttagtgaagcctggagggtccctgaaactctcctgtgcagcctctggattcactttcagtagctatgacatgtcttgggttcgccagactccggagaagagtctggagtgggtcgcaaccattagtgatggtggtggttacatctactattcagacagtgtgaaggggcgatttaccatctccagagacaatgccaagaacaacctgtacctgcaaatgagcagtctgaggtctgaggacacggccttgtatatttgtgcaagagaatttggtaagcgctatgctttggactactggggtcaaggaacctcagtcaccgtctcctca

SEQ ID NO: 113 - protein, 116 aa, synthetic construct
  REGION 1..116: note = Synthetic
EVKLVESGGDLVKPGGSLKLSCAASGFTFSSYDMSWVRQTPEKSLEWVATISDGGGYIYYSDSVKGRFTISRDNAKNNLYLQMSSLRSEDTALYICAREFGKRYALDYWGQGTSVT

SEQ ID NO: 114 - DNA, 321 bp, synthetic construct
  misc_feature 1..321: note = Synthetic
  source 1..321: mol_type = other DNA
gacattgtgatgacccagtctcacaaattcatgtccacatcggtaggagacagggtcagcatctcctgcaaggccagtcaggatgtgactcctgctgtcgcctggtatcaacagaagccaggacaatctcctaaactactgatttactccacatcctcccggtacactggagtccctgatcgcttcactggcagtggatctgggacggatttcactttcaccatcagcagtgtgcaggctgaagacctggcagtttattactgtcagcaacattatactactccgctcacgttcggtgctgggaccaagctggagctgaaa

SEQ ID NO: 115 - protein, 107 aa, synthetic construct; identical to SEQ ID NO: 27
  REGION 1..107: note = Synthetic

SEQ ID NO: 116 - protein, 5 aa, synthetic construct
  REGION 1..5: note = Synthetic
SYAIS

SEQ ID NO: 117 - protein, 5 aa, synthetic construct
  REGION 1..5: note = Synthetic
SYAMS

SEQ ID NO: 118 - protein, 17 aa, synthetic construct
  REGION 1..17: note = Synthetic
GIIPIFGTANYAQKFQG

SEQ ID NO: 119 - protein, 17 aa, synthetic construct
  REGION 1..17: note = Synthetic
AISGSGGSTYYADSVKG

SEQ ID NO: 120 - protein, 9 aa, synthetic construct
  REGION 1..9: note = Synthetic
ARGSSWFDY

SEQ ID NO: 121 - protein, 12 aa, synthetic construct
  REGION 1..12: note = Synthetic
ASSYHGGGYHRY

SEQ ID NO: 122 - protein, 12 aa, synthetic construct
  REGION 1..12: note = Synthetic
TTSKYSGSALRY

SEQ ID NO: 123 - protein, 10 aa, synthetic construct
  REGION 1..10: note = Synthetic
ARDRTGAFDY

SEQ ID NO: 124 - protein, 12 aa, synthetic construct
  REGION 1..12: note = Synthetic
ARHETVAGSFDY

SEQ ID NO: 125 - protein, 15 aa, synthetic construct
  REGION 1..15: note = Synthetic
ARTGYYGGNSGAFDI

SEQ ID NO: 126 - protein, 13 aa, synthetic construct
  REGION 1..13: note = Synthetic
ARAGTGMDLVFNS

SEQ ID NO: 127 - protein, 13 aa, synthetic construct
  REGION 1..13: note = Synthetic
ARGLARGDLNFGY

SEQ ID NO: 128 - protein, 8 aa, synthetic construct
  REGION 1..8: note = Synthetic
TREPHFDY

SEQ ID NO: 129 - protein, 14 aa, synthetic construct
  REGION 1..14: note = Synthetic
TTAAPGSYYLVFHY

SEQ ID NO: 130 - protein, 14 aa, synthetic construct
  REGION 1..14: note = Synthetic
ARDAGPVGYYGMDV

SEQ ID NO: 131 - protein, 13 aa, synthetic construct
  REGION 1..13: note = Synthetic
AGDGLYGSGSFGY

SEQ ID NO: 132 - protein, 12 aa, synthetic construct
  REGION 1..12: note = Synthetic
AKDIRWFYGMDV

SEQ ID NO: 133 - protein, 14 aa, synthetic construct
  REGION 1..14: note = Synthetic
ARHESGIAGGHFDY

SEQ ID NO: 134 - protein, 12 aa, synthetic construct
  REGION 1..12: note = Synthetic
AKDIRWYYGMDV

SEQ ID NO: 135 - protein, 17 aa, synthetic construct
  REGION 1..17: note = Synthetic
AKGVRGTYQIGYYGMDV

SEQ ID NO: 136 - protein, 11 aa, synthetic construct
  REGION 1..11: note = Synthetic
ARQGTAMALDY

SEQ ID NO: 137 - protein, 14 aa, synthetic construct
  REGION 1..14: note = Synthetic
VRDLQDWNYGGAAY

SEQ ID NO: 138 - protein, 12 aa, synthetic construct
  REGION 1..12: note = Synthetic
ARDDYYYGQFDS

SEQ ID NO: 139 - protein, 14 aa, synthetic construct
  REGION 1..14: note = Synthetic
AREITGTSYTALDS

SEQ ID NO: 140 - protein, 13 aa, synthetic construct
  REGION 1..13: note = Synthetic
ARGHIDGQAAGDY

SEQ ID NO: 141 - protein, 12 aa, synthetic construct
  REGION 1..12: note = Synthetic
AASTLRVPNPPY

SEQ ID NO: 142 - protein, 13 aa, synthetic construct
  REGION 1..13: note = Synthetic
ARSGDRYDFWSGY

SEQ ID NO: 143 - protein, 14 aa, synthetic construct
  REGION 1..14: note = Synthetic
TRGQDSTWYSSFDY

SEQ ID NO: 144 - protein, 12 aa, synthetic construct
  REGION 1..12: note = Synthetic
AASTLRLPNPPY

SEQ ID NO: 145 - protein, 14 aa, synthetic construct
  REGION 1..14: note = Synthetic
ATTQTSFYSHGMDV

SEQ ID NO: 146 - protein, 14 aa, synthetic construct
  REGION 1..14: note = Synthetic
ARVRKTPFWGALDS

SEQ ID NO: 147 - protein, 13 aa, synthetic construct
  REGION 1..13: note = Synthetic
ARGFTYGDFIFDY

SEQ ID NO: 148 - protein, 14 aa, synthetic construct
  REGION 1..14: note = Synthetic
ARDVRGVTYLGMDV

SEQ ID NO: 149 - protein, 14 aa, synthetic construct
  REGION 1..14: note = Synthetic
ARVRKTPFWGTLDS

SEQ ID NO: 150 - protein, 14 aa, synthetic construct
  REGION 1..14: note = Synthetic
ARVRRTPFWGALDS

SEQ ID NO: 151 - protein, 18 aa, synthetic construct
  REGION 1..18: note = Synthetic
AKRKGLGSPTDYYYGMDV

SEQ ID NO: 152 - protein, 14 aa, synthetic construct
  REGION 1..14: note = Synthetic
VRPEYDTYYYGMDV

SEQ ID NO: 153 - protein, 9 aa, synthetic construct
  REGION 1..9: note = Synthetic
AKGGGSYDY

SEQ ID NO: 154 - protein, 9 aa, synthetic construct
  REGION 1..9: note = Synthetic
ARALNGMDV

SEQ ID NO: 155 - protein, 20 aa, synthetic construct
  REGION 1..20: note = Synthetic
TRPLQGIAAADSYYYYAMDV

SEQ ID NO: 156 - protein, 13 aa, synthetic construct
  REGION 1..13: note = Synthetic
ARLHSYLSEEFDP

SEQ ID NO: 157 - protein, 12 aa, synthetic construct
  REGION 1..12: note = Synthetic
AKLSAVNTYIDD

SEQ ID NO: 158 - protein, 14 aa, synthetic construct
  REGION 1..14: note = Synthetic
ARVTKTPFWGTLDY

SEQ ID NO: 159 - protein, 14 aa, synthetic construct
  REGION 1..14: note = Synthetic
ARVSQSPVWGYFDY

SEQ ID NO: 160 - protein, 15 aa, synthetic construct
  REGION 1..15: note = Synthetic
AKDGYYDFWSGYSDY

SEQ ID NO: 161 - protein, 11 aa, synthetic construct
  REGION 1..11: note = Synthetic
QANQDIHHYLN

SEQ ID NO: 162 - protein, 17 aa, synthetic construct
  REGION 1..17: note = Synthetic
KSSQSVLYSSSNKNYLA

SEQ ID NO: 163 - protein, 17 aa, synthetic construct
  REGION 1..17: note = Synthetic
KSSQSVLYSSNNKNYLA

SEQ ID NO: 164 - protein, 16 aa, synthetic construct
  REGION 1..16: note = Synthetic
RSSQNLLHSDGYNYLN

SEQ ID NO: 165 - protein, 17 aa, synthetic construct
  REGION 1..17: note = Synthetic
KSSQSVLYTSNNKNYLA

SEQ ID NO: 166 - protein, 11 aa, synthetic construct
  REGION 1..11: note = Synthetic
QASQDINRYLS

SEQ ID NO: 167 - protein, 11 aa, synthetic construct
  REGION 1..11: note = Synthetic
QASQDISNYLN

SEQ ID NO: 168 - protein, 11 aa, synthetic construct
  REGION 1..11: note = Synthetic
RASQTISSHLN

SEQ ID NO: 169 - protein, 11 aa, synthetic construct
  REGION 1..11: note = Synthetic
RASQGIAGWLA

SEQ ID NO: 170 - protein, 11 aa, synthetic construct
  REGION 1..11: note = Synthetic
RASQGVSSWLA

SEQ ID NO: 171 - protein, 17 aa, synthetic construct
  REGION 1..17: note = Synthetic
KSSQSLFYHSNNHNYLA

SEQ ID NO: 172 - protein, 11 aa, synthetic construct
  REGION 1..11: note = Synthetic
RASQGISSSLA

SEQ ID NO: 173 - protein, 11 aa, synthetic construct
  REGION 1..11: note = Synthetic
QASRDISNSLS

SEQ ID NO: 174 - protein, 11 aa, synthetic construct
  REGION 1..11: note = Synthetic
RASQSISRYLN

SEQ ID NO: 175 - protein, 11 aa, synthetic construct
  REGION 1..11: note = Synthetic
RASRSISNWLA

SEQ ID NO: 176 - protein, 17 aa, synthetic construct
  REGION 1..17: note = Synthetic
KSSQSVFYRSNQKNYLA

SEQ ID NO: 177 - protein, 11 aa, synthetic construct
  REGION 1..11: note = Synthetic
RASQSVSSYLA

SEQ ID NO: 178 - protein, 11 aa, synthetic construct
  REGION 1..11: note = Synthetic
RASRGISSWLA

SEQ ID NO: 179 - protein, 11 aa, synthetic construct
  REGION 1..11: note = Synthetic
RASQGISSWLA

SEQ ID NO: 180 - protein, 11 aa, synthetic construct
  REGION 1..11: note = Synthetic
RASQSISSYLN

SEQ ID NO: 181 - protein, 11 aa, synthetic construct
  REGION 1..11: note = Synthetic
RASQAISNLLA

SEQ ID NO: 182 - protein, 11 aa, synthetic construct
  REGION 1..11: note = Synthetic
RASQGISTWLA

SEQ ID NO: 183 - protein, 11 aa, synthetic construct
  REGION 1..11: note = Synthetic
RASQGIASNLA

SEQ ID NO: 184 - protein, 11 aa, synthetic construct
  REGION 1..11: note = Synthetic
RASQGVSSYLA

SEQ ID NO: 185 - protein, 11 aa, synthetic construct
  REGION 1..11: note = Synthetic
RASQSIYTYLN

SEQ ID NO: 186 - protein, 11 aa, synthetic construct
  REGION 1..11: note = Synthetic
RASQFVSDWLA

SEQ ID NO: 187 - protein, 11 aa, synthetic construct
  REGION 1..11: note = Synthetic
RASQTISTWLA

SEQ ID NO: 188 - protein, 11 aa, synthetic construct
  REGION 1..11: note = Synthetic
RASQGISSYLA

SEQ ID NO: 189 - protein, 11 aa, synthetic construct
  REGION 1..11: note = Synthetic
RASQSIGYWLA

SEQ ID NO: 190 - protein, 11 aa, synthetic construct
  REGION 1..11: note = Synthetic
RATQSISSWLA

SEQ ID NO: 191 - protein, 11 aa, synthetic construct
  REGION 1..11: note = Synthetic
RASQGVRNWLA

SEQ ID NO: 192 - protein, 11 aa, synthetic construct
  REGION 1..11: note = Synthetic
RASQSINNYLA

SEQ ID NO: 193 - protein, 11 aa, synthetic construct
  REGION 1..11: note = Synthetic
RASQDITSWLA

SEQ ID NO: 194 - protein, 11 aa, synthetic construct
  REGION 1..11: note = Synthetic
RASQGIYDYLA

SEQ ID NO: 195 - protein, 11 aa, synthetic construct
  REGION 1..11: note = Synthetic
RASEGISGWLA

SEQ ID NO: 196 - protein, 7 aa, synthetic construct
  REGION 1..7: note = Synthetic
DASILQS

SEQ ID NO: 197 - protein, 7 aa, synthetic construct
  REGION 1..7: note = Synthetic
WASTRES

SEQ ID NO: 198 - protein, 7 aa, synthetic construct
  REGION 1..7: note = Synthetic
LGSNRAT

SEQ ID NO: 199 - protein, 7 aa, synthetic construct
  REGION 1..7: note = Synthetic
DASNLET

SEQ ID NO: 200 - protein, 7 aa, synthetic construct
  REGION 1..7: note = Synthetic
AASSLQS

SEQ ID NO: 201 - protein, 7 aa, synthetic construct
  REGION 1..7: note = Synthetic
AASTLQS

SEQ ID NO: 202 - protein, 7 aa, synthetic construct
  REGION 1..7: note = Synthetic
AAFSLQS

SEQ ID NO: 203 - protein, 7 aa, synthetic construct
  REGION 1..7: note = Synthetic
GASSRAT

SEQ ID NO: 204 - protein, 7 aa, synthetic construct
  REGION 1..7: note = Synthetic
GISSRAT

SEQ ID NO: 205 - protein, 7 aa, synthetic construct
  REGION 1..7: note = Synthetic
AVSTLQS

SEQ ID NO: 206 - protein, 7 aa, synthetic construct
  REGION 1..7: note = Synthetic
DISTLQN

SEQ ID NO: 207 - protein, 7 aa, synthetic construct
  REGION 1..7: note = Synthetic
GASTLQS

SEQ ID NO: 208 - protein, 7 aa, synthetic construct
  REGION 1..7: note = Synthetic
GASSLQS

SEQ ID NO: 209 - protein, 7 aa, synthetic construct
  REGION 1..7: note = Synthetic
AASTLES

SEQ ID NO: 210 - protein, 7 aa, synthetic construct
  REGION 1..7: note = Synthetic
DASSLQS

SEQ ID NO: 211 - protein, 7 aa, synthetic construct
  REGION 1..7: note = Synthetic
KASNLQS

SEQ ID NO: 212 - protein, 7 aa, synthetic construct
  REGION 1..7: note = Synthetic
TASTLQN

SEQ ID NO: 213 - protein, 7 aa, synthetic construct
  REGION 1..7: note = Synthetic
RASSLQS

SEQ ID NO: 214 - protein, 7 aa, synthetic construct
  REGION 1..7: note = Synthetic
AASHLQS

SEQ ID NO: 215 - protein, 7 aa, synthetic construct
  REGION 1..7: note = Synthetic
DASTLQS

SEQ ID NO: 216 - protein, 7 aa, synthetic construct
  REGION 1..7: note = Synthetic
AASNLER

SEQ ID NO: 217 - protein, 7 aa, synthetic construct
  REGION 1..7: note = Synthetic
AASSLET

SEQ ID NO: 218 - protein, 9 aa, synthetic construct
  REGION 1..9: note = Synthetic
QQADSFPIT

SEQ ID NO: 219 - protein, 9 aa, synthetic construct
  REGION 1..9: note = Synthetic
QQSYSTPWT

SEQ ID NO: 220 - protein, 9 aa, synthetic construct
  REGION 1..9: note = Synthetic
QQYYSTPWT

SEQ ID NO: 221 - protein, 9 aa, synthetic construct
  REGION 1..9: note = Synthetic
QQSFTTPWT

SEQ ID NO: 222 - protein, 9 aa, synthetic construct
  REGION 1..9: note = Synthetic
QQYDNLPPT

SEQ ID NO: 223 - protein, 9 aa, synthetic construct
  REGION 1..9: note = Synthetic
QQSYGSPVT

SEQ ID NO: 224 - protein, 9 aa, synthetic construct
  REGION 1..9: note = Synthetic
QQGNSFPFT

SEQ ID NO: 225 - protein, 9 aa, synthetic construct
  REGION 1..9: note = Synthetic
QQAKSFPLT

SEQ ID NO: 226 - protein, 9 aa, synthetic construct
  REGION 1..9: note = Synthetic
QQVKSFPLT

SEQ ID NO: 227 - protein, 9 aa, synthetic construct
  REGION 1..9: note = Synthetic
QQYYNTPWT

SEQ ID NO: 228 - protein, 9 aa, synthetic construct
  REGION 1..9: note = Synthetic
QQTKNFPLT

SEQ ID NO: 229 - protein, 11 aa, synthetic construct
  REGION 1..11: note = Synthetic
RASQDIVNWLA

SEQ ID NO: 230 - protein, 9 aa, synthetic construct
  REGION 1..9: note = Synthetic
QQTKSFPLT

SEQ ID NO: 231 - protein, 9 aa, synthetic construct
  REGION 1..9: note = Synthetic
QQSYNTPRT

SEQ ID NO: 232 - protein, 9 aa, synthetic construct
  REGION 1..9: note = Synthetic
QQSYRAPWT

SEQ ID NO: 233 - protein, 9 aa, synthetic construct
  REGION 1..9: note = Synthetic
QQANNFPLT

SEQ ID NO: 234 - protein, 9 aa, synthetic construct
  REGION 1..9: note = Synthetic
QQGNSFPLT

SEQ ID NO: 235 - protein, 9 aa, synthetic construct
  REGION 1..9: note = Synthetic
QQSKNFPVT

SEQ ID NO: 236 - protein, 9 aa, synthetic construct
  REGION 1..9: note = Synthetic
QQANSFPLT

SEQ ID NO: 237 - protein, 9 aa, synthetic construct
  REGION 1..9: note = Synthetic
QQLESYPLT

SEQ ID NO: 238 - protein, 8 aa, synthetic construct
  REGION 1..8: note = Synthetic
QQYYSSPT

SEQ ID NO: 239 - protein, 9 aa, synthetic construct
  REGION 1..9: note = Synthetic
QQLKTFPLT

SEQ ID NO: 240 - protein, 9 aa, synthetic construct
  REGION 1..9: note = Synthetic
QQTNWFPLT

SEQ ID NO: 241 - protein, 9 aa, synthetic construct
  REGION 1..9: note = Synthetic
QQAQSFPIT

SEQ ID NO: 242 - protein, 9 aa, synthetic construct
  REGION 1..9: note = Synthetic
QQAHSFPLT

SEQ ID NO: 243 - protein, 9 aa, synthetic construct
  REGION 1..9: note = Synthetic
LQDYHFPLT

SEQ ID NO: 244 - protein, 9 aa, synthetic construct
  REGION 1..9: note = Synthetic
QQGHSFPLT

SEQ ID NO: 245 - protein, 9 aa, synthetic construct
  REGION 1..9: note = Synthetic
QQSYIFPLT

SEQ ID NO: 246 - protein, 8 aa, synthetic construct
  REGION 1..8: note = Synthetic
QQYDTYWT

SEQ ID NO: 247 - protein, 10 aa, synthetic construct
  REGION 1..10: note = Synthetic
QQLNSYPLFT

SEQ ID NO: 248 - protein, 8 aa, synthetic construct
  REGION 1..8: note = Synthetic
QQYSSYWT

SEQ ID NO: 249 - protein, 9 aa, synthetic construct
  REGION 1..9: note = Synthetic
LQHNTYPFT

SEQ ID NO: 250 - protein, 9 aa, synthetic construct
  REGION 1..9: note = Synthetic
QQGHSFPLT

SEQ ID NO: 251 - protein, 9 aa, synthetic construct
  REGION 1..9: note = Synthetic
QQAHSFPFT

SEQ ID NO: 252 - protein, 9 aa, synthetic construct
  REGION 1..9: note = Synthetic
QQANMFPLT

SEQ ID NO: 253 - protein, 9 aa, synthetic construct
  REGION 1..9: note = Synthetic
QQADSFPFT

SEQ ID NO: 254 - protein, 116 aa, synthetic construct
  REGION 1..116: note = Synthetic
QVQLVQSGAEVKKPGSSVKVSCKASGGTFSSYAISWVRQAPGQGLEWMGGIIPIFGTANYAQKFQGRVTITADESTSTAYMELSSLRSEDTAVYYCARGSSWFDYWGQGTLVTVSS

SEQ ID NO: 255 - protein, 119 aa, synthetic construct
  REGION 1..119: note = Synthetic
QVQLVQSGAEVKKPGSSVKVSCKASGGTFSSYAISWVRQAPGQGLEWMGGIIPIFGTANYAQKFQGRVTITADESTSTAYMELSSLRSEDTAVYYCASSYHGGGYHRYWGQGTLVTVSS

SEQ ID NO: 256 - protein, 119 aa, synthetic construct
  REGION 1..119: note = Synthetic
QVQLVQSGAEVKKPGSSVKVSCKASGGTFSSYAISWVRQAPGQGLEWMGGIIPIFGTANYAQKFQGRVTITADESTSTAYMELSSLRSEDTAVYYCTTSKYSGSALRYWGQGTLVTVSS

SEQ ID NO: 257 - protein, 117 aa, synthetic construct
  REGION 1..117: note = Synthetic
QVQLVQSGAEVKKPGSSVKVSCKASGGTFSSYAISWVRQAPGQGLEWMGGIIPIFGTANYAQKFQGRVTITADESTSTAYMELSSLRSEDTAVYYCARDRTGAFDYWGQGTLVTVSS

SEQ ID NO: 258 - protein, 119 aa, synthetic construct
  REGION 1..119: note = Synthetic
QVQLVQSGAEVKKPGSSVKVSCKASGGTFSSYAISWVRQAPGQGLEWMGGIIPIFGTANYAQKFQGRVTITADESTSTAYMELSSLRSEDTAVYYCARHETVAGSFDYWGQGTLVTVSS

SEQ ID NO: 259 - protein, 122 aa, synthetic construct
  REGION 1..122: note = Synthetic
QVQLVQSGAEVKKPGSSVKVSCKASGGTFSSYAISWVRQAPGQGLEWMGGIIPIFGTANYAQKFQGRVTITADESTSTAYMELSSLRSEDTAVYYCARTGYYGGNSGAFDIWGQGTMVTVSS

SEQ ID NO: 260 - protein, 120 aa, synthetic construct
  REGION 1..120: note = Synthetic
QVQLVQSGAEVKKPGSSVKVSCKASGGTFSSYAISWVRQAPGQGLEWMGGIIPIFGTANYAQKFQGRVTITADESTSTAYMELSSLRSEDTAVYYCARAGTGMDLVFNSWGQGTLVTVSS

SEQ ID NO: 261 - protein, 120 aa, synthetic construct
  REGION 1..120: note = Synthetic
QVQLVQSGAEVKKPGSSVKVSCKASGGTFSSYAISWVRQAPGQGLEWMGGIIPIFGTANYAQKFQGRVTITADESTSTAYMELSSLRSEDTAVYYCARGLARGDLNFGYWGQGTLVTVSS

SEQ ID NO: 262 - protein, 115 aa, synthetic construct
  REGION 1..115: note = Synthetic
QVQLVQSGAEVKKPGSSVKVSCKASGGTFSSYAISWVRQAPGQGLEWMGGIIPIFGTANYAQKFQGRVTITADESTSTAYMELSSLRSEDTAVYYCTREPHFDYWGQGTLVTVSS

SEQ ID NO: 263 - protein, 121 aa, synthetic construct
  REGION 1..121: note = Synthetic
QVQLVQSGAEVKKPGSSVKVSCKASGGTFSSYAISWVRQAPGQGLEWMGGIIPIFGTANYAQKFQGRVTITADESTSTAYMELSSLRSEDTAVYYCTTAAPGSYYLVFHYWGQGTLVTVSS

SEQ ID NO: 264 - protein, 121 aa, synthetic construct
  REGION 1..121: note = Synthetic
QVQLVQSGAEVKKPGSSVKVSCKASGGTFSSYAISWVRQAPGQGLEWMGGIIPIFGTANYAQKFQGRVTITADESTSTAYMELSSLRSEDTAVYYCARDAGPVGYYGMDVWGQGTTVTVSS

SEQ ID NO: 265 - protein, 120 aa, synthetic construct
  REGION 1..120: note = Synthetic
QVQLVQSGAEVKKPGSSVKVSCKASGGTFSSYAISWVRQAPGQGLEWMGGIIPIFGTANYAQKFQGRVTITADESTSTAYMELSSLRSEDTAVYYCAGDGLYGSGSFGYWGQGTPVTVSS

SEQ ID NO: 266 - protein, 120 aa, synthetic construct
  REGION 1..120: note = Synthetic
QVQLVQSGAEVKKPGSSVKVSCKASGGTFSSYAISWVRQAPGQGLEWMGGIIPIFGTANYAQKFQGRVTITADESTSTAYMELSSLRSEDTAVYYCAKDIRWFYGMDVWGQGTTVTVSSW

SEQ ID NO: 267 - protein, 121 aa, synthetic construct
  REGION 1..121: note = Synthetic
QVQLVQSGAEVKKPGSSVKVSCKASGGTFSSYAISWVRQAPGQGLEWMGGIIPIFGTANYAQKFQGRVTITADESTSTAYMELSSLRSEDTAVYYCARHESGIAGGHFDYWGQGTLVTVSS

SEQ ID NO: 268 - protein, 120 aa, synthetic construct
  REGION 1..120: note = Synthetic
QVQLVQSGAEVKKPGSSVKVSCKASGGTFSSYAISWVRQAPGQGLEWMGGIIPIFGTANYAQKFQGRVTITADESTSTAYMELSSLRSEDTAVYYCARDAGPVGYYGMDVWGQGTTVTVS

SEQ ID NO: 269 - protein, 119 aa, synthetic construct
  REGION 1..119: note = Synthetic
QVQLVQSGAEVKKPGSSVKVSCKASGGTFSSYAISWVRQAPGQGLEWMGGIIPIFGTANYAQKFQGRVTITADESTSTAYMELSSLRSEDTAVYYCAKDIRWYYGMDVWGQGTTVTVSS

SEQ ID NO: 270 - protein, 124 aa, synthetic construct
  REGION 1..124: note = Synthetic
QVQLVQSGAEVKKPGSSVKVFCKASGGTFSSYAISWVRQAPGQGLEWMGGIIPIFGTANYAQKFQGRVTITADESTSTAYMELSSLRSEDTAVYYCAKGVRGTYQIGYYGMDVWGQGTTVTVSS

SEQ ID NO: 271 - protein, 118 aa, synthetic construct
  REGION 1..118: note = Synthetic
QVQLVQSGAEVKKPGSSVKVSCKASGGTFSSYAISWVRQAPGQGLEWMGGIIPIFGTANYAQKFQGRVTITADESTSTAYMELSSLRSEDTAVYYCARQGTAMALDYWGQGTLVTVSS

SEQ ID NO: 272 - protein, 121 aa, synthetic construct
  REGION 1..121: note = Synthetic
QVQLVQSGAEVKKPGSSVKVSCKASGGTFSSYAISWVRQAPGQGLEWMGGIIPIFGTANYAQKFQGRVTITADESTSTAYMELSSLRSEDTAVYYCVRDLQDWNYGGAAYWGQGTLVTVSS

SEQ ID NO: 273 - protein, 119 aa, synthetic construct
  REGION 1..119: note = Synthetic
QVQLVQSGAEVKKPGSSVKVSCKASGGTFSSYAISWVRQAPGQGLEWMGGIIPIFGTANYAQKFQGRVTITADESTSTAYMELSSLRSEDTAVYYCARDDYYYGQFDSWGQGTLVTVSS

SEQ ID NO: 274 - protein, 121 aa, synthetic construct
  REGION 1..121: note = Synthetic
QVQLVQSGAEVKKPGSSVKVSCKASGGTFSSYAISWVRQAPGQGLEWMGGIIPIFGTANYAQKFQGRVTITADESTSTAYMELSSLRSEDTAVYYCAREITGTSYTALDSWGQGTLVTVSS

SEQ ID NO: 275 - protein, 120 aa, synthetic construct
  REGION 1..120: note = Synthetic
QVQLVQSGAEVKKPGSSVKVSCKASGGTFSSYAISWVRQAPGQGLEWMGGIIPIFGTANYAQKFQGRVTITADESTSTAYMELSSLRSEDTAVYYCARGHIDGQAAGDYWGQGTLVTVSS

SEQ ID NO: 276 - protein, 119 aa, synthetic construct
  REGION 1..119: note = Synthetic
QVQLVQSGAEVKKPGSSVKVSCKASGGTFSSYAISWVRQAPGQGLEWMGGIIPIFGTANYAQKFQGRVTITADESTSTAYMELSSLRSEDTAVYYCAASTLRVPNPPYWGQGTLVTVSS

SEQ ID NO: 277 - protein, 120 aa, synthetic construct
  REGION 1..120: note = Synthetic
QVQLVQSGAEVKKPGSSVKVSCKASGGTFSSYAISWVRQAPGQGLEWMGGIIPIFGTANYAQKFQGRVTITADESTSTAYMELSSLRSEDTAVYYCARSGDRYDFWSGYWGQGTLVTVSS

SEQ ID NO: 278 - protein, 119 aa, synthetic construct; identical to SEQ ID NO: 276
  REGION 1..119: note = Synthetic

SEQ ID NO: 279 - protein, 121 aa, synthetic construct
  REGION 1..121: note = Synthetic
QVQLVQSGAEVKKPGSSVKVSCKASGGTFSSYAISWVRQAPGQGLEWMGGIIPIFGTANYAQKFQGRVTITADESTSTAYMELSSLRSEDTAVYYCARDAGPVGYYGMDVWGQGTMVTVSS

SEQ ID NO: 280 - protein, 121 aa, synthetic construct
  REGION 1..121: note = Synthetic
QVQLVQSGAEVKKPGSSVKVSCKASGGTFSSYAISWVRQAPGQGLEWMGGIIPIFGTANYAQKFQGRVTITADESTSTAYMELSSLRSEDTAVYYCTRGQDSTWYSSFDYWGQGTLVTVSS

SEQ ID NO: 281 - protein, 119 aa, synthetic construct
  REGION 1..119: note = Synthetic
QVQLVQSGAEVKKPGSSVKVSCKASGGTFSSYAISWVRQAPGQGLEWMGGIIPIFGTANYAQKFQGRVTITADESTSTAYMELSSLRSEDTAVYYCAASTLRLPNPPYWGQGTLVTVSS

SEQ ID NO: 282 - protein, 121 aa, synthetic construct
  REGION 1..121: note = Synthetic
QVQLVQSGAEVKKPGSSVKVSCKASGGTFSSYAISWVRQAPGQGLEWMGGIIPIFGTANYAQKFQGRVTITADESTSTAYMELSSLRSEDTAVYYCATTQTSFYSHGMDVWGQGTTVTVSS

SEQ ID NO: 283 - protein, 119 aa, synthetic construct
  REGION 1..119: note = Synthetic
QLLESGGGLVQPGGSLRLSCAASGFTFSSYAMSWVRQAPGKGLEWVSAISGSGGSTYYADSVKGRFTISRDNSKNTLYLQMNSLRAEDTAVYYCARVRKTPFWGALDSWGRGTLVTVSS

SEQ ID NO: 284 - protein, 120 aa, synthetic construct
  REGION 1..120: note = Synthetic
QVQLVQSGAEVKKPGSSVKVSCKASGGTFSSYAISWVRQAPGQGLEWMGGIIPIFGTANYAQKFQGRVTITADESTSTAYMELSSLRSEDTAVYYCARGFTYGDFIFDYWGQGTLVTVSS

SEQ ID NO: 285 - protein, 121 aa, synthetic construct
  REGION 1..121: note = Synthetic
QVQLVQSGAEVKKPGSSVKVSCKASGGTFSSYAISWVRQAPGQGLEWMGGIIPIFGTANYAQKFQGRVTITADESTSTAYMELSSLRSEDTAVYYCARDVRGVTYLGMDVWGQGTTVTVSS

SEQ ID NO: 286 - protein, 119 aa, synthetic construct
  REGION 1..119: note = Synthetic
QLLESGGGLVQPGGSLRLSCAASGFTFSSYAMSWVRQAPGKGLEWVSAISGSGGSTYYADSVKGRFTISRDNSKNTLYLQMNSLRAEDTAVYYCARVRKTPFWGTLDSWGRGTLVTVSS

SEQ ID NO: 287 - protein, 119 aa, synthetic construct
  REGION 1..119: note = Synthetic
QLLESGGGLVQPGGSLRLSCAASGFTFSSYAMSWVRQAPGKGLEWVSAISGSGGSTYYADSVKGRFTISRDNSKNTLYLQMNSLRAEDTAVYYCARVRRTPFWGALDSWGRGTLVTVSS

SEQ ID NO: 288 - protein, 119 aa, synthetic construct; identical to SEQ ID NO: 283
  REGION 1..119: note = Synthetic

SEQ ID NO: 289 - protein, 123 aa, synthetic construct
  REGION 1..123: note = Synthetic
QLLESGGGLVQPGGSLRLSCAASGFTFSSYAMSWVRQAPGKGLEWVSAISGSGGSTYYADSVKGRFTISRDNSKNTLYLQMNSLRAEDTAVYYCAKRKGLGSPTDYYYGMDVWGQGTTVTVSS

SEQ ID NO: 290 - protein, 119 aa, synthetic construct; identical to SEQ ID NO: 283
  REGION 1..119: note = Synthetic

SEQ ID NO: 291 - protein, 119 aa, synthetic construct
  REGION 1..119: note = Synthetic
QLLESGGGLVQPGGSLRLSCAASGFTFSSYAMSWVRQAPGKGLEWVSAISGSGGSTYYADSVKGRFTISRDNSKNTLYLQMNSLRAEDTAVYYCARVRKTPFWGTLDSWGRGSLVTVSS

SEQ ID NO: 292 - protein, 119 aa, synthetic construct
  REGION 1..119: note = Synthetic
QLLESGGGLVQPGGSLRLSCAASGFTFSSYAMSWVRQAPGKGLEWVSAISGSGGSTYYADSVKGRFTISRDNSKNTLYLQMNSLRAEDTAVYYCVRPEYDTYYYGMDVWGQGTTVTVSS

SEQ ID NO: 293 - protein, 114 aa, synthetic construct
  REGION 1..114: note = Synthetic
QLLESGGGLVQPGGSLRLSCAASGFTFSSYAMSWVRQAPGKGLEWVSAISGSGGSTYYADSVKGRFTISRDNSKNTLYLQMNSLRAEDTAVYYCAKGGGSYDYWGQGTLVTVSS

SEQ ID NO: 294 - protein, 114 aa, synthetic construct
  REGION 1..114: note = Synthetic
QLLESGGGLVQPGGSLRLSCAASGFTFSSYAMSWVRQAPGKGLEWVSAISGSGGSTYYADSVKGRFTISRDNSKNTLYLQMNSLRAEDTAVYYCARALNGMDVWGQGTMVTVSS

SEQ ID NO: 295 - protein, 125 aa, synthetic construct
  REGION 1..125: note = Synthetic
QLLESGGGLVQPGGSLRLSCAASGFTFSSYAMSWVRQAPGKGLEWVSAISGSGGSTYYADSVKGRFTISRDNSKNTLYLQMNSLRAEDTAVYYCTRPLQGIAAADSYYYYAMDVWGQGTTVTVSS

SEQ ID NO: 296 - protein, 118 aa, synthetic construct
  REGION 1..118: note = Synthetic
QLLESGGGLVQPGGSLRLSCAASGFTFSSYAMSWVRQAPGKGLEWVSAISGSGGSTYYADSVKGRFTISRDNSKNTLYLQMNSLRAEDTAVYYCARLHSYLSEEFDPWGQGTLVTVSS

SEQ ID NO: 297 - protein, 119 aa, synthetic construct; identical to SEQ ID NO: 283
  REGION 1..119: note = Synthetic

SEQ ID NO: 298 - protein, 117 aa, synthetic construct
  REGION 1..117: note = Synthetic
QLLESGGGLVQPGGSLRLSCAASGFTFSSYAMSWVRQAPGKGLEWVSAISGSGGSTYYADSVKGRFTISRDNSKNTLYLQMNSLRAEDTAVYYCAKLSAVNTYIDDWGQGTLVTVSS

SEQ ID NO: 299 - protein, 119 aa, synthetic construct
  REGION 1..119: note = Synthetic
QLLESGGGLVQPGGSLRLSCAASGFTFSSYAMSWVRQAPGKGLEWVSAISGSGGSTYYADSVKGRFTISRDNSKNTLYLQMNSLRAEDTAVYYCARVTKTPFWGTLDYWGQGTLVTVSS

SEQ ID NO: 300 - protein, 119 aa, synthetic construct; identical to SEQ ID NO: 287
  REGION 1..119: note = Synthetic

SEQ ID NO: 301 - protein, 119 aa, synthetic construct
  REGION 1..119: note = Synthetic
QLLESGGGLVQPGGSLRLSCAASGFTFSSYAMSWVRQAPGKGLEWVSAISGSGGSTYYADSVKGRFTISRDNSKNTLYLQMNSLRAEDTAVYYCARVSQSPVWGYFDYWGQGMLVTVSS

SEQ ID NO: 302 - protein, 120 aa, synthetic construct
  REGION 1..120: note = Synthetic
QLLESGGGLVQPGGSLRLSCAASGFTFSSYAMSWVRQAPGKGLEWVSAISGSGGSTYYADSVKGRFTISRDNSKNTLYLQMNSLRAEDTAVYYCAKDGYYDFWSGYSDYWGQGTLVTVSS

SEQ ID NO: 303 - protein, 108 aa, synthetic construct
  REGION 1..108: note = Synthetic
DIQLTQSPSSLSAFVGDRVTITCQANQDIHHYLNWYQQKPGKAPKLLIYDASILQSGVPSRFSGSGSGTDFTLTISSLQPEDFATYFCQQADSFPITFGQGTRLEIKR

SEQ ID NO: 304 - protein, 114 aa, synthetic construct
  REGION 1..114: note = Synthetic
EIVLTQSPDSLAVSLGERATINCKSSQSVLYSSSNKNYLAWYQQKPGQPPKLLIYWASTRESGVPDRFSGSGSGTDFTLTISSLQPEDFATYYCQQSYSTPWTFGPGTKLEIKR

SEQ ID NO: 305 - protein, 114 aa, synthetic construct
  REGION 1..114: note = Synthetic
DIQMTQSPDSLAVSLGERATINCKSSQSVLYSSNNKNYLAWYQQKPGHPPKLLVYWASTRESGVPARFSASGSGTDFTLAISNLQAEDVAVYYCQQYYSTPWTFGQGTKVEIKR

SEQ ID NO: 306 - protein, 113 aa, synthetic construct
  REGION 1..113: note = Synthetic
EIVLTQSPLSLPVTPGEPASISCRSSQNLLHSDGYNYLNWYLQKPGQSPQLLIYLGSNRATGVPDRFSGSGSGTDFTLTISSLQPEDFATYYCQQSYSTPWTFGQGTKVEIKR

SEQ ID NO: 307 - protein, 114 aa, synthetic construct
  REGION 1..114: note = Synthetic
DIVMTQSPDSLAVSLGERATINCKSSQSVLYTSNNKNYLAWYQQKPGQPPKLLIYWASTRESGVPDRFSGSGSGTDFTLTISSLQAEDVAIYYCQQYYSTPWTFGQGTKLEIKR

SEQ ID NO: 308 - protein, 114 aa, synthetic construct
  REGION 1..114: note = Synthetic
AIQLTQSPDSLAVSLGERATINCKSSQSVLYSSNNKNYLAWYQQKPGQPPKLLIYWASTRESGVPDRFSGSGSGTDFTLTISSLQAEDSATYYCQQSFTTPWTFGQGTKVEIKR

SEQ ID NO: 309 - protein, 108 aa, synthetic construct
  REGION 1..108: note = Synthetic
DIQMTQSPSSLSASVGDRVTITCQASQDINRYLSWYQQKPGKAPKLLIYDASNLETGVPSRFSGSASGTDFTFAISSLQPEDIATYYCQQYDNLPPTFGQGTRLEIKR

SEQ ID NO: 310 - protein, 108 aa, synthetic construct
  REGION 1..108: note = Synthetic
EIVMTQSPSSLSASVGDRVTITCQASQDISNYLNWYQQKPGKAPKLLIYAASSLQSGVPSRFSGSGSGTDFTLTISSLQPEDFASYYCQQSYGSPVTFGQGTKLEIKR

SEQ ID NO: 311 - protein, 108 aa, synthetic construct
  REGION 1..108: note = Synthetic
EIVMTQSPSSLSASVGDRVTITCQASQDISNYLNWYQQKPGKAPKLLIYDASNLETGVPSRFSGSGSGTEFTLTISSLRPEDFATYFCQQADSFPITFGQGTRLEIKR

SEQ ID NO: 312 - protein, 108 aa, synthetic construct
  REGION 1..108: note = Synthetic
DIQLTQSPSSLSASVGDRVTITCRASQTISSHLNWYQQKPGKAPKVLIYAASSLQSGVPSRFSGSGSGTEFTLTISSLQPDDFATYYCQQGNSFPFTFGPGTKVEIKR

SEQ ID NO: 313 - protein, 108 aa, synthetic construct
  REGION 1..108: note = Synthetic
AIRMTQSPSTLSASVGDRVTITCRASQGIAGWLAWYQQKPGKAPKLLIYAASSLQSGVPSRFSGSASGTDFTLTISNLQPEDFATYYCQQAKSFPLTFGGGTKVEIKR

SEQ ID NO: 314 - protein, 113 aa, synthetic construct
  REGION 1..113: note = Synthetic
DIVMTQSPDSLAVSLGERATINCKSSQSVLYSSNNKNYLAWYQQKPGQPPKLLIYWASTRESGVPDRFSGTGSGTDFTLTISSLQAEDVAVYYCQQSYSTPWTFGQGTKLEIK

SEQ ID NO: 315 - protein, 108 aa, synthetic construct
  REGION 1..108: note = Synthetic
DIVMTQSPSSVSAFVGDRVTITCRASQGVSSWLAWFQQKPGKAPKLLIYAASTLQSGVPSRFSGRGYGTEFTLTISSLQPEDLATYYCQQVKSFPLTFGGGTKVDIKR

SEQ ID NO: 316 - protein, 114 aa, synthetic construct
  REGION 1..114: note = Synthetic
DIVMTQSPDSLAVSLGERATINCKSSQSLFYHSNNHNYLAWYQQKPGQPPKLLIYWASTRQSGVPDRFTGSGSGTDFTLTISSLQAEDVAVYYCQQYYNTPWTFGQGTKVEIKR

SEQ ID NO: 317 - protein, 108 aa, synthetic construct; identical to SEQ ID NO: 313
  REGION 1..108: note = Synthetic

SEQ ID NO: 318 - protein, 108 aa, synthetic construct; identical to SEQ ID NO: 315
  REGION 1..108: note = Synthetic

SEQ ID NO: 319 - protein, 108 aa, synthetic construct
  REGION 1..108: note = Synthetic
DIVMTQSPSSLSASVGDRVTITCRASQGISSSLAWYQQKPGKAPNLLIYTASTLQNGVPSRFSGSGSGTDFTLTISGLQPEDFATYYCQQTKNFPLTFGQGTRLEIKR

SEQ ID NO: 320 - protein, 114 aa, synthetic construct
  REGION 1..114: note = Synthetic
EIVLTQSPDSLAVSLGERATINCKSSQSVLYSSNNKNYLAWYQQRPGQPPKLLISWASTRESGVPDRFSGSGSGADFSLTISSLQAEDVAVYYCQQYYSTPWTFGQGTKLEIKR

SEQ ID NO: 321 - protein, 108 aa, synthetic construct
  REGION 1..108: note = Synthetic
VIWMTQSPSSLSASVGDSVTITCQASRDISNSLSWHQQKPGKAPKLLIYAASSLQSGVPSRFSGSGSGTDFTLTISSLQPEDFATYYCQQTKSFPLTFGGGTKVEIKR

SEQ ID NO: 322 - protein, 108 aa, synthetic construct
  REGION 1..108: note = Synthetic
EIVMTQSPSSLSASVGDRVTISCRASQSISRYLNWYQQKPGQAPKLLIYAAFSLQSGVPSRFSGSGSGTDFTLTISSLQPEDFATYYCQQSYNTPRTFGQGTKLEIKR

SEQ ID NO: 323 - protein, 107 aa, synthetic construct
  REGION 1..107: note = Synthetic
DVVMTQSPSTVSASVGDRITITCRASRSISNWLAWYQQKPGKAPKLLIYAASSLQSGVPSRFSGSGSGTDFTLTISSLQPEDFATYYCQQAKSFPLTFGGGTKVEIK

SEQ ID NO: 324 - protein, 114 aa, synthetic construct
  REGION 1..114: note = Synthetic
DIQLTQSPDSLAVSLGERATINCKSSQSVFYRSNQKNYLAWYQQKPGQTPRLLIYGASSRATGIPDRFSGSGSGTDFTLTISSLQPEDFATYYCQQSYRAPWTFGQGTKVEIKR

SEQ ID NO: 325 - protein, 108 aa, synthetic construct
  REGION 1..108: note = Synthetic
EIVLTQSPGTLSLSPGERATLSCRASQSVSSYLAWYQQKPGQAPRLLIYGISSRATGIPDRFSGSGSGTDFTLTISSLQPEDFATYYCQQANNFPLTFGGGTKLEIKR

SEQ ID NO: 326 - protein, 108 aa, synthetic construct
  REGION 1..108: note = Synthetic
EIVLTQSPSSVSASVGDRVTITCRASRGISSWLAWYQQKPGKAPKLLIYAASTLQSGVPSRFSGSGSGTDFTLTISSLQPEDFATYYCQQAKSFPLTFGGGTKVEIKR

SEQ ID NO: 327 - protein, 108 aa, synthetic construct; identical to SEQ ID NO: 325
  REGION 1..108: note = Synthetic

SEQ ID NO: 328 - protein, 108 aa, synthetic construct
  REGION 1..108: note = Synthetic
AIQMTQSPSSLSASVGDRVTITCRASQGISSWLAWYQQKPGKAPKLLIYAASSLQSGVPSRFSGSGSGTDFTLTISRLQPEDFATYYCQQAKSFPLTFGGGTKVEIKR

SEQ ID NO: 329 - protein, 108 aa, synthetic construct
  REGION 1..108: note = Synthetic
AIRMTQSPSSLSASVGDRVTITCRASQSISSYLNWYQQKPGKAPNLLIYAVSTLQSGVPSRFSGSGSGTVFTLTISSLQPEDFATYFCQQGNSFPLTFGGGTKVEIKR

SEQ ID NO: 330 - protein, 108 aa, synthetic construct
  REGION 1..108: note = Synthetic
DIQLTQSPSTLSASVGDRVTITCRASQAISNLLAWYQQKPGKPPNLLIYDISTLQNGVPSRFSGSGSGTDFTLTINSLQPEDFAIYYCQQSKNFPVTFGGGTKVEIKR

SEQ ID NO: 331 - protein, 108 aa, synthetic construct
  REGION 1..108: note = Synthetic
DIQLTQSPSSVSASVGDRVTITCRASQGISSWLAWYQQKPGKAPKLLIYGASTLQSGVPSRFSGSGSGADYTLTISSLQPEDFATYYCQQANSFPLTFAGGTKLEIKR

SEQ ID NO: 332 - protein, 108 aa, synthetic construct
  REGION 1..108: note = Synthetic
DIQLTQSPSSLSASPGDRVTITCRASQGISTWLAWYQQKPGNAPKLLIYAASSLQSGVPSRFSGSKSGTEYTLTISSLQPEDFATYYCQQLESYPLTFGGGTKVEIKR

SEQ ID NO: 333 - protein, 113 aa, synthetic construct
  REGION 1..113: note = Synthetic
AIRMTQSPDSLVVSLGERATINCKSSQSVLYSSNNKNYLAWYQQKPGQPPKLLIYWASTRESGVPDRFSGSGSGTDFTLSISSLQAEDVAVYYCQQYYSSPTFGGGTKVEIKR

SEQ ID NO: 334 - protein, 108 aa, synthetic construct
  REGION 1..108: note = Synthetic
DVVMTQSPFFLSASVGDRVTITCRASQGIASNLAWYQQKPGKAPKLLIYAASTLQSGVPSRFTGSGSGTEFTLTVTSLQPEDFATYYCQQLKTFPLTFGGGTKVEIKR

SEQ ID NO: 335 - protein, 108 aa, synthetic construct
  REGION 1..108: note = Synthetic
VIWMTQSPSSLSASVGDRVTITCRASQGVSSYLAWYQQKPGKAPKLLIYAASSLQSGVPSRFSGSGSGTEFTLTISSLQPEDFATYYCQQTNWFPLTFGPGTRLEIKR

SEQ ID NO: 336 - protein, 108 aa, synthetic construct
  REGION 1..108: note = Synthetic
DIQMTQSPSSLSTSAGDTVTITCRASQSIYTYLNWYQQKPGKAPNLLIYGASSLQSGVPSRFSGSGSGTDFTLTISSLQPEDFATYYCQQAQSFPITFGQGTRLEIKR

SEQ ID NO: 337 - protein, 108 aa, synthetic construct
  REGION 1..108: note = Synthetic
VIWMTQSPSSVSASVGDRVTITCRASQGISSWLAWYQQKPGKAPKLLIYAASSLQSGVPSRFSGSGSGTDFTLTISSLQPEDFATYYCQQAHSFPLTFGGGTKVEIKR

SEQ ID NO: 338 - protein, 108 aa, synthetic construct
  REGION 1..108: note = Synthetic
AIQLTQSPSTLSASVGDRVTITCRASQFVSDWLAWYQQKPGKAPKLLIYAASTLQSGVPSRFSGSGSGTDFTLTISSLQPEDLATYYCLQDYHFPLTFGGGTKLEIKR

SEQ ID NO: 339 - protein, 108 aa, synthetic construct
  REGION 1..108: note = Synthetic
DVVMTQSPSSVSASVGDRVTITCRASQDIVNWLAWYQQKPGKAPKLLIYAASTLESGAPSRFSASGSGTDFTLTISSLQPDDFATYYCQQGHSFPLTFGPGTKLEIKR

SEQ ID NO: 340 - protein, 108 aa, synthetic construct
  REGION 1..108: note = Synthetic
DIVMTQSPSSLSASVGDRVTITCRASQSIYTYLNWYQQKPGKAPKLLIYDASSLQSGVPSRFSGSGYGTEFTLTISGLQPEDFATYYCQQSYIFPLTFGRGTKVEIKR

SEQ ID NO: 341 - protein, 107 aa, synthetic construct
  REGION 1..107: note = Synthetic
AIRMTQSPSFVSASVGDRVTIACRASQTISTWLAWYQQKPGKAPKVLISKASNLQSGVPSRFSGSGSGTEFTLTISSLQPDDFATYYCQQYDTYWTFGQGTKVEIKR

SEQ ID NO: 342 - protein, 107 aa, synthetic construct; identical to SEQ ID NO: 341
  REGION 1..107: note = Synthetic

SEQ ID NO: 343 - protein, 109 aa, synthetic construct
  REGION 1..109: note = Synthetic
DIVMTQSPSFVSASVGDTVTITCRASQGISSYLAWYQQKPGKAPKLLIYAASTLQSGVPSRFSGSGSGTEFTLTISSLQPEDFATYYCQQLNSYPLFTFGPGTKVEIKR

SEQ ID NO: 344 - protein, 107 aa, synthetic construct
  REGION 1..107: note = Synthetic
DIQMTQSPSTLSASVGDRVTITCRASQSIGYWLAWYQQKPGKAPKLLIYRASSLQSGVPSRFSGSGSATEFTLTITSLQPDDFATYFCQQYSSYWTFGQGTKVEIKR

SEQ ID NO: 345 - protein, 108 aa, synthetic construct
  REGION 1..108: note = Synthetic
EIVLTQSPSSLSASVGDTVTITCRATQSISSWLAWYQQKPGKAPQRLISGASTLQSGVPSRFSGSGSGTEFTLTISGLQPEDFATYYCLQHNTYPFTFGQGTKVEIKR

SEQ ID NO: 346 - protein, 108 aa, synthetic construct
  REGION 1..108: note = Synthetic
DIVMTQSPSSVSASVGDRVTITCRASQGVRNWLAWYQQKPGKAPKLLIYAASHLQSGVPSRFSGSGSGTDFTLTISSLQTDDFATYYCQQGHSFPLTFGGGTKVEIKR

SEQ ID NO: 347 - protein, 108 aa, synthetic construct; identical to SEQ ID NO: 346
  REGION 1..108: note = Synthetic

SEQ ID NO: 348 - protein, 108 aa, synthetic construct
  REGION 1..108: note = Synthetic
VIWMTQSPSTLSASVGDRVTITCRASQSINNYLAWYQQKPGKAPKLLIYDASTLQSGVPSRFSGGGSGTDFTLTINSLQPDDFASYYCQQAHSFPFTFGGGTKLEIKR

SEQ ID NO: 349 - protein, 108 aa, synthetic construct
  REGION 1..108: note = Synthetic
EIVMTQSPSSVSASVGDRVTITCRASQDITSWLAWYQQKPGKAPKLLIYAASTLESGVPSRFSGSGSGTDFTLTITGLQPEDFATYYCQQANMFPLTFGGGTKVEIKR

SEQ ID NO: 350 - protein, 108 aa, synthetic construct
  REGION 1..108: note = Synthetic
AIRMTQSPSSLSASVGDRVTITCRASQGIYDYLAWYQQKPGKAPSLLIYAASNLERGVPSRFSGSGSGKYFILTISSLQPEDFATYYCQQANSFPLTFGGGTKVEIKR

SEQ ID NO: 351 - protein, 108 aa, synthetic construct
  REGION 1..108: note = Synthetic
AIQLTQSPSSLSASVGDRVTITCRASEGISGWLAWYQQIPGKAPKLLIYAASSLETGVPSRFSGSGYGTDFTLTISSLQPEDFATYYCQQADSFPFTFGPGTKVEIKR

SEQ ID NO: 352 - protein, 116 aa, synthetic construct
  REGION 1..116: note = Synthetic
QVQLQQSGSELVRPGTSVKISCKASGYTFTNYWLGWIKQRPGHGLEWIGDIYPGGDYINYNEKFKGKATLSADTSSSTAYMQLSSLTSEDSAVYFCARPNLPGDYWGQGTSVTVSS

SEQ ID NO: 353 - protein, 112 aa, synthetic construct
  REGION 1..112: note = Synthetic
DIVMTQAAFSNPVTLGTSASISCRSSKSLLHSNGITYLYWYLQKPGQSPQLLIYQVSNLASGVPGRFSGSGSGTDFTLRISRVEAEDVGVYYCAQNLELPWTFGGGTKLEIK

SEQ ID NO: 354 - protein, 10 aa, synthetic construct
  REGION 1..10: note = Synthetic
GYTFTNYWLG

SEQ ID NO: 355 - protein, 17 aa, synthetic construct
  REGION 1..17: note = Synthetic
DIYPGGDYINYNEKFKG

SEQ ID NO: 356 - protein, 7 aa, synthetic construct
  REGION 1..7: note = Synthetic
PNLPGDY

SEQ ID NO: 357 - protein, 16 aa, synthetic construct
  REGION 1..16: note = Synthetic
RSSKSLLHSNGITYLY

SEQ ID NO: 358 - protein, 7 aa, synthetic construct
  REGION 1..7: note = Synthetic
QVSNLAS

SEQ ID NO: 359 - protein, 9 aa, synthetic construct
  REGION 1..9: note = Synthetic
AQNLELPWT

SEQ ID NO: 360 - protein, 116 aa, synthetic construct
  REGION 1..116: note = Synthetic
QVQLVQSGAEVKKPGASVKVSCKASGYTFTNYWLGWVRQAPGQGLEWMGDIYPGGDYINYNEKFKGRVTMTRDTSISTAYMELSRLRSDDTAVYYCARPNLPGDYWGQGTTVTVSS

SEQ ID NO: 361 - protein, 116 aa, synthetic construct
  REGION 1..116: note = Synthetic
QVQLVQSGAEVKKPGASVKVSCKASGYTFTNYWLGWVRQAPGQGLEWMGDIYPGGDYINYNEKFKGRVTMTADTSISTAYMELSRLRSDDTAVYYCARPNLPGDYWGQGTTVTVSS

SEQ ID NO: 362 - protein, 116 aa, synthetic construct
  REGION 1..116: note = Synthetic
QVQLVQSGAEVKKPGASVKVSCKASGYTFTNYWLGWVRQAPGQGLEWMGDIYPGGDYINYNEKFKGRVTLTADTSISTAYMELSRLRSDDTAVYYCARPNLPGDYWGQGTTVTVSS

SEQ ID NO: 363 - protein, 116 aa, synthetic construct
  REGION 1..116: note = Synthetic
QVQLVQSGAEVKKPGASVKVSCKASGYTFTNYWLGWVRQAPGQGLEWMGDIYPGGDYINYNEKFKGKATLTADTSISTAYMELSRLRSDDTAVYYCARPNLPGDYWGQGTTVTVSS

SEQ ID NO: 364 - protein, 116 aa, synthetic construct
  REGION 1..116: note = Synthetic
QVQLVQSGAEVKKPGASVKVSCKASGYTFTNYWLGWVRQAPGQGLEWIGDIYPGGDYINYNEKFKGKATLTADTSISTAYMELSRLRSDDTAVYYCARPNLPGDYWGQGTTVTVSS

SEQ ID NO: 365 - protein, 116 aa, synthetic construct
  REGION 1..116: note = Synthetic
QVQLVQSGAEVKKPGASVKVSCKASGYTFTNYWLGWIKQAPGQGLEWIGDIYPGGDYINYNEKFKGKATLTADTSISTAYMELSRLRSDDTAVYYCARPNLPGDYWGQGTTVTVSS

SEQ ID NO: 366 - protein, 116 aa, synthetic construct
  REGION 1..116: note = Synthetic
QVQLVQSGAEVKKPGASVKVSCKASGYTFTNYWLGWIKQAPGQGLEWIGDIYPGGDYINYNEKFKGKATLTADTSISTAYMELSRLRSDDTAVYFCARPNLPGDYWGQGTTVTVSS

SEQ ID NO: 367 - protein, 116 aa, synthetic construct
  REGION 1..116: note = Synthetic
EVQLVQSGAEVKKPGASVKVSCKASGYTFTNYWLGWVRQAPGQGLEWMGDIYPGGDYINYNEKFKGRVTMTRDTSISTAYMELSRLRSDDTAVYYCARPNLPGDYWGQGTTVTVSS

SEQ ID NO: 368 - protein, 116 aa, synthetic construct
  REGION 1..116: note = Synthetic
EVQLVQSGAEVKKPGASVKVSCKASGYTFTNYWLGWVRQAPGQGLEWMGDIYPGGDYINYNEKFKGRVTMTADTSISTAYMELSRLRSDDTAVYYCARPNLPGDYWGQGTTVTVSS

SEQ ID NO: 369 - protein, 116 aa, synthetic construct
  REGION 1..116: note = Synthetic
EVQLVQSGAEVKKPGASVKVSCKASGYTFTNYWLGWVRQAPGQGLEWMGDIYPGGDYINYNEKFKGRVTLTADTSISTAYMELSRLRSDDTAVYYCARPNLPGDYWGQGTTVTVSS

SEQ ID NO: 370 - protein, 116 aa, synthetic construct
  REGION 1..116: note = Synthetic
EVQLVQSGAEVKKPGASVKVSCKASGYTFTNYWLGWVRQAPGQGLEWMGDIYPGGDYINYNEKFKGKATLTADTSISTAYMELSRLRSDDTAVYYCARPNLPGDYWGQGTTVTVSS

SEQ ID NO: 371 - protein, 116 aa, synthetic construct
  REGION 1..116: note = Synthetic
EVQLVQSGAEVKKPGASVKVSCKASGYTFTNYWLGWVRQAPGQGLEWIGDIYPGGDYINYNEKFKGKATLTADTSISTAYMELSRLRSDDTAVYYCARPNLPGDYWGQGTTVTVSS

SEQ ID NO: 372 - protein, 116 aa, synthetic construct
  REGION 1..116: note = Synthetic
EVQLVQSGAEVKKPGASVKVSCKASGYTFTNYWLGWIKQAPGQGLEWIGDIYPGGDYINYNEKFKGKATLTADTSISTAYMELSRLRSDDTAVYYCARPNLPGDYWGQGTTVTVSS

SEQ ID NO: 373 - protein, 116 aa, synthetic construct
  REGION 1..116: note = Synthetic
EVQLVQSGAEVKKPGASVKVSCKASGYTFTNYWLGWIKQAPGQGLEWIGDIYPGGDYINYNEKFKGKATLTADTSISTAYMELSRLRSDDTAVYFCARPNLPGDYWGQGTTVTVSS

SEQ ID NO: 374 - protein, 112 aa, synthetic construct
  REGION 1..112: note = Synthetic
DIVMTQSPLSLPVTPGEPASISCRSSKSLLHSNGITYLYWYLQKPGQSPQLLIYQVSNLASGVPDRFSGSGSGTDFTLKISRVEAEDVGVYYCAQNLELPWTFGGGTKVEIK

SEQ ID NO: 375 - protein, 116 aa, synthetic construct
  REGION 1..116: note = Synthetic
EVQLVQSGAEVKKPGASVKVSCKASGYTFTNYWLGWIKQAPGQGLEWIGDIYPGGDYINYNEKFKGKATLTADTSISTAYMELSRLRSDDTAVYYCARPNLPKDHWGQGTTVTVSS

SEQ ID NO: 376 - protein, 112 aa, synthetic construct
  REGION 1..112: note = Synthetic
DIVMTQSPLSLPVTPGEPASISCRSSKSLLHSNAITYLYWYLQKPGQSPQLLIYQVSNLASGVPDRFSGSGSGTDFTLKISRVEAEDVGVYYCAQNLELPWTFGGGTKVEIK

SEQ ID NO: 377 - protein, 116 aa, synthetic construct
  REGION 1..116: note = Synthetic
EVQLVQSGAEVKKPGASVKVSCKASGYTFTNYWLGWIKQAPGQGLEWIGDIYPGGDYINYNEKFKGKATLTADTSISTAYMELSRLRSDDTAVYYCARPDLPGDYWGQGTTVTVSS

SEQ ID NO: 378 - protein, 112 aa, synthetic construct; identical to SEQ ID NO: 376
  REGION 1..112: note = Synthetic

SEQ ID NO: 379 - protein, 116 aa, synthetic construct
  REGION 1..116: note = Synthetic
EVQLVQSGAEVKKPGASVKVSCKASGYTFTNYWLGWIKQAPGQGLEWIGDIYPGGDYINYNEKFKGKATLTADTSISTAYMELSRLRSDDTAVYYCARPGLPKDYWGQGTTVTVSS

SEQ ID NO: 380 - protein, 112 aa, synthetic construct; identical to SEQ ID NO: 376
  REGION 1..112: note = Synthetic

SEQ ID NO: 381 - protein, 116 aa, synthetic construct
  REGION 1..116: note = Synthetic
EVQLVQSGAEVKKPGASVKVSCKASGYTFTNYWLGWIKQAPGQGLEWIGDIYPGGDYINYNEKFKGKATLTADTSISTAYMELSRLRSDDTAVYYCARPNLPKDYWGQGTTVTVSS

SEQ ID NO: 382 - protein, 112 aa, synthetic construct; identical to SEQ ID NO: 376
  REGION 1..112: note = Synthetic

SEQ ID NO: 383 - protein, 116 aa, synthetic construct
  REGION 1..116: note = Synthetic
EVQLVQSGAEVKKPGASVKVSCKASGYTFTNYWLGWIKQAPGQGLEWIGDIYPGGDYINYNEKFKGKATLTADTSISTAYMELSRLRSDDTAVYYCARPNLPRDYWGQGTTVTVSS

SEQ ID NO: 384 - protein, 112 aa, synthetic construct; identical to SEQ ID NO: 376
  REGION 1..112: note = Synthetic

SEQ ID NO: 385 - protein, 116 aa, synthetic construct
  REGION 1..116: note = Synthetic
EVQLVQSGAEVKKPGASVKVSCKASGYTFTNYWLGWIKQAPGQGLEWIGDIYPGGDYINYNEKFKGKATLTADTSISTAYMELSRLRSDDTAVYYCARPGLPRDYWGQGTTVTVSS

SEQ ID NO: 386 - protein, 112 aa, synthetic construct; identical to SEQ ID NO: 376
  REGION 1..112: note = Synthetic

SEQ ID NO: 387 - protein, 116 aa, synthetic construct
  REGION 1..116: note = Synthetic
EVQLVQSGAEVKKPGASVKVSCKASGYTFTNYWLGWIKQAPGQGLEWIGDIYPGGDYINYNEKFKGKATLTADTSISTAYMELSRLRSDDTAVYYCARPGLPQDYWGQGTTVTVSS

SEQ ID NO: 388 - protein, 112 aa, synthetic construct; identical to SEQ ID NO: 376
  REGION 1..112: note = Synthetic

SEQ ID NO: 389 - protein, 116 aa, synthetic construct
  REGION 1..116: note = Synthetic
EVQLVQSGAEVKKPGASVKVSCKASGYTFTNYWLGWIKQAPGQGLEWIGDIYPGGDYINYNEKFKGKATLTADTSISTAYMELSRLRSDDTAVYYCARPDLPKDYWGQGTTVTVSS

SEQ ID NO: 390 - protein, 112 aa, synthetic construct; identical to SEQ ID NO: 376
  REGION 1..112: note = Synthetic

SEQ ID NO: 391 - protein, 116 aa, synthetic construct; identical to SEQ ID NO: 372
  REGION 1..116: note = Synthetic

SEQ ID NO: 392 - protein, 112 aa, synthetic construct
  REGION 1..112: note = Synthetic
DIVMTQSPLSLPVTPGEPASISCRSSKSLLHSNAITYLYWYLQKPGQSPQLLIYQVSNLASGVPDRFSGSGSGTDFTLKISRVEAEDVGVYYCGQNLELPWTFGGGTKVEIK

SEQ ID NO: 393 - protein, 116 aa, synthetic construct; identical to SEQ ID NO: 372
  REGION 1..116: note = Synthetic

SEQ ID NO: 394 - protein, 112 aa, synthetic construct
  REGION 1..112: note = Synthetic
DIVMTQSPLSLPVTPGEPASISCRSSKSLLHSNAITYLYWYLQKPGQSPQLLIYQVSNLASGVPDRFSGSGSGTDFTLKISRVEAEDVGVYYCAQNLEMPWTFGGGTKVEIK

SEQ ID NO: 395 - protein, 116 aa, synthetic construct; identical to SEQ ID NO: 372
  REGION 1..116: note = Synthetic

SEQ ID NO: 396 - protein, 112 aa, synthetic construct
  REGION 1..112: note = Synthetic
DIVMTQSPLSLPVTPGEPASISCRSSKSLLHSNAITYLYWYLQKPGQSPQLLIYQVSNLASGVPDRFSGSGSGTDFTLKISRVEAEDVGVYYCGQNLEMPWTFGGGTKVEIK

SEQ ID NO: 397 - protein, 116 aa, synthetic construct; identical to SEQ ID NO: 372
  REGION 1..116: note = Synthetic

SEQ ID NO: 398 - protein, 112 aa, synthetic construct
  REGION 1..112: note = Synthetic
DIVMTQSPLSLPVTPGEPASISCRSSKSLLHSNAITYLYWYLQKPGQSPQLLIYQVSNLASGVPDRFSGSGSGTDFTLKISRVEAEDVGVYYCAQYLEEPWTFGGGTKVEIK

SEQ ID NO: 399 - protein, 116 aa, synthetic construct; identical to SEQ ID NO: 372
  REGION 1..116: note = Synthetic

SEQ ID NO: 400 - protein, 112 aa, synthetic construct
  REGION 1..112: note = Synthetic
DIVMTQSPLSLPVTPGEPASISCRSSKSLLHSNAITYLYWYLQKPGQSPQLLIYQVSNLASGVPDRFSGSGSGTDFTLKISRVEAEDVGVYYCAQYLELPWTFGGGTKVEIK

SEQ ID NO: 401 - protein, 116 aa, synthetic construct; identical to SEQ ID NO: 375
  REGION 1..116: note = Synthetic

SEQ ID NO: 402 - protein, 112 aa, synthetic construct; identical to SEQ ID NO: 392
  REGION 1..112: note = Synthetic

SEQ ID NO: 403 - protein, 116 aa, synthetic construct; identical to SEQ ID NO: 375
  REGION 1..116: note = Synthetic

SEQ ID NO: 404 - protein, 112 aa, synthetic construct; identical to SEQ ID NO: 398
  REGION 1..112: note = Synthetic

SEQ ID NO: 405 - protein, 116 aa, synthetic construct; identical to SEQ ID NO: 375
  REGION 1..116: note = Synthetic

SEQ ID NO: 406 - protein, 112 aa, synthetic construct; identical to SEQ ID NO: 400
  REGION 1..112: note = Synthetic

SEQ ID NO: 407 - protein, 116 aa, synthetic construct
  REGION 1..116: note = Synthetic
EVQLVQSGAEVKKPGASVKVSCKASGYTFENYWLGWIKQAPGQGLEWIGDIYPGGDYIVYNEKFKGKATLTADTSISTAYMELSRLRSDDTAVYYCARPNLPGDYWGQGTTVTVSS

SEQ ID NO: 408 - protein, 112 aa, synthetic construct
  REGION 1..112: note = Synthetic
DIVMTQSPLSLPVTPGEPASISCRSSKSLLHSNAITYLYWYLQKPGQSPQLLIYQVSNLARGVPDRFSGSGSGTDFTLKISRVEAEDVGVYYCAQNLELPWTFGGGTKVEIK

SEQ ID NO: 409 - protein, 116 aa, synthetic construct
  REGION 1..116: note = Synthetic
EVQLVQSGAEVKKPGASVKVSCKASGYMFTNYWLGWIKQAPGQGLEWIGDIYPGGDYINYNEKFKGKATLTADTSISTAYMELSRLRSDDTAVYYCARPNLPGDYWGQGTTVTVSS

SEQ ID NO: 410 - protein, 112 aa, synthetic construct
  REGION 1..112: note = Synthetic
DIVMTQSPLSLPVTPGEPASISCRSSKSLLHSNAITYLYWYLQKPGQSPQLLIYQKSNLASGVPDRFSGSGSGTDFTLKISRVEAEDVGVYYCAQNLELPWTFGGGTKVEIK

SEQ ID NO: 411 - protein, 116 aa, synthetic construct
  REGION 1..116: note = Synthetic
EVQLVQSGAEVKKPGASVKVSCKASGYTFDNYWLGWIKQAPGQGLEWIGDIYPGGDIINYNEKFKGKATLTADTSISTAYMELSRLRSDDTAVYYCARPNLPGDYWGQGTTVTVSS

SEQ ID NO: 412 - protein, 112 aa, synthetic construct
  REGION 1..112: note = Synthetic
DIVMTQSPLSLPVTPGEPASISCRSSKSLLHSNAITYLYWYLQKPGQSPQLLIYQVSNLAVGVPDRFSGSGSGTDFTLKISRVEAEDVGVYYCAQNLELPWTFGGGTKVEIK

SEQ ID NO: 413 - protein, 116 aa, synthetic construct
  REGION 1..116: note = Synthetic
EVQLVQSGAEVKKPGASVKVSCKASGYTFGNYWLGWIKQAPGQGLEWIGDIYPGGDVINYNEKFKGKATLTADTSISTAYMELSRLRSDDTAVYYCARPNLPGDYWGQGTTVTVSS

SEQ ID NO: 414 - protein, 112 aa, synthetic construct
  REGION 1..112: note = Synthetic
DIVMTQSPLSLPVTPGEPASISCRSSKSLLHSNAITYLYWYLQKPGQSPQLLIYQVSNLALGVPDRFSGSGSGTDFTLKISRVEAEDVGVYYCAQNLELPWTFGGGTKVEIK

SEQ ID NO: 415 - protein, 116 aa, synthetic construct
  REGION 1..116: note = Synthetic
EVQLVQSGAEVKKPGASVKVSCKASGYTFTNYWLWWIKQAPGQGLEWIGDIFPGGDYINYNEKFKGKATLTADTSISTAYMELSRLRSDDTAVYYCARPNLPGDYWGQGTTVTVSS

SEQ ID NO: 416 - protein, 112 aa, synthetic construct
  REGION 1..112: note = Synthetic
DIVMTQSPLSLPVTPGEPASISCRSSKSLLHSNAITYLYWYLQKPGQSPQLLIYQVDNLASGVPDRFSGSGSGTDFTLKISRVEAEDVGVYYCAQNLELPWTFGGGTKVEIK

SEQ ID NO: 417 - protein, 116 aa, synthetic construct
  REGION 1..116: note = Synthetic
EVQLVQSGAEVKKPGASVKVSCKASGYTFTNYWLGWIKQAPGQGLEWIGDIYPGGDYIVYNEKFKGKATLTADTSISTAYMELSRLRSDDTAVYYCARPNLPGDYWGQGTTVTVSS

SEQ ID NO: 418 - protein, 112 aa, synthetic construct
  REGION 1..112: note = Synthetic
DIVMTQSPLSLPVTPGEPASISCRSSKSLLHSNAITYLYWYLQKPGQSPQLLIYQVSNLATGVPDRFSGSGSGTDFTLKISRVEAEDVGVYYCAQNLELPWTFGGGTKVEIK

SEQ ID NO: 419 - protein, 116 aa, synthetic construct
  REGION 1..116: note = Synthetic
EVQLVQSGAEVKKPGASVKVSCKASGYLFTNYWLGWIKQAPGQGLEWIGDIYPGGDYIVYNEKFKGKATLTADTSISTAYMELSRLRSDDTAVYYCARPNLPGDYWGQGTTVTVSS

SEQ ID NO: 420 - protein, 112 aa, synthetic construct; identical to SEQ ID NO: 376
  REGION 1..112: note = Synthetic

SEQ ID NO: 421 - protein, 116 aa, synthetic construct; identical to SEQ ID NO: 372
  REGION 1..116: note = Synthetic

SEQ ID NO: 422 - protein, 112 aa, synthetic construct
  REGION 1..112: note = Synthetic
DIVMTQSPLSLPVTPGEPASISCRSSKSLLHSNAITYLYWYLQKPGQSPQLLIYHVSNLASGVPDRFSGSGSGTDFTLKISRVEAEDVGVYYCAQNLELPWTFGGGTKVEIK

SEQ ID NO: 423 - protein, 116 aa, synthetic construct
  REGION 1..116: note = Synthetic
EVQLVQSGAEVKKPGASVKVSCKASGYTFTNYWLWWIKQAPGQGLEWIGDIYPGGDLINYNEKFKGKATLTADTSISTAYMELSRLRSDDTAVYYCARPNLPGDYWGQGTTVTVSS

SEQ ID NO: 424 - protein, 112 aa, synthetic construct; identical to SEQ ID NO: 422
  REGION 1..112: note = Synthetic

SEQ ID NO: 425 - protein, 116 aa, synthetic construct
  REGION 1..116: note = Synthetic
EVQLVQSGAEVKKPGASVKVSCKASGYTFTNYWLSWIKQAPGQGLEWIGDIYPGGDHINYNEKFKGKATLTADTSISTAYMELSRLRSDDTAVYYCARPNLPGDYWGQGTTVTVSS

SEQ ID NO: 426 - protein, 112 aa, synthetic construct; identical to SEQ ID NO: 376
  REGION 1..112: note = Synthetic

SEQ ID NO: 427 - protein, 116 aa, synthetic construct
  REGION 1..116: note = Synthetic
EVQLVQSGAEVKKPGASVKVSCKASGYTFTNYWLWWIKQAPGQGLEWIGEIYPGGDYITYNEKFKGKATLTADTSISTAYMELSRLRSDDTAVYYCARPNLPGDYWGQGTTVTVSS

SEQ ID NO: 428 - protein, 112 aa, synthetic construct
  REGION 1..112: note = Synthetic
DIVMTQSPLSLPVTPGEPASISCRSSKSLLHSNAITYLYWYLQKPGQSPQLLIYQVSNRASGVPDRFSGSGSGTDFTLKISRVEAEDVGVYYCAQNLELPWTFGGGTKVEIK

SEQ ID NO: 429 - protein, 116 aa, synthetic construct; identical to SEQ ID NO: 372
  REGION 1..116: note = Synthetic

SEQ ID NO: 430 - protein, 112 aa, synthetic construct; identical to SEQ ID NO: 416
  REGION 1..112: note = Synthetic

SEQ ID NO: 431 - protein, 116 aa, synthetic construct
  REGION 1..116: note = Synthetic
EVQLVQSGAEVKKPGASVKVSCKASGFTFTNYWLGWIKQAPGQGLEWIGDIYPGGDYIVYNEKFKGKATLTADTSISTAYMELSRLRSDDTAVYYCARPNLPGDYWGQGTTVTVSS

SEQ ID NO: 432 - protein, 112 aa, synthetic construct; identical to SEQ ID NO: 376
  REGION 1..112: note = Synthetic

SEQ ID NO: 433 - protein, 116 aa, synthetic construct; identical to SEQ ID NO: 375
  REGION 1..116: note = Synthetic

SEQ ID NO: 434 - protein, 112 aa, synthetic construct; identical to SEQ ID NO: 418
  REGION 1..112: note = Synthetic

SEQ ID NO: 435 - protein, 116 aa, synthetic construct; identical to SEQ ID NO: 417
  REGION 1..116: note = Synthetic

SEQ ID NO: 436 - protein, 112 aa, synthetic construct; identical to SEQ ID NO: 392
  REGION 1..112: note = Synthetic

SEQ ID NO: 437 - protein, 116 aa, synthetic construct; identical to SEQ ID NO: 417
  REGION 1..116: note = Synthetic

SEQ ID NO: 438 - protein, 112 aa, synthetic construct; identical to SEQ ID NO: 400
  REGION 1..112: note = Synthetic

SEQ ID NO: 439 - protein, 116 aa, synthetic construct; identical to SEQ ID NO: 419
  REGION 1..116: note = Synthetic

SEQ ID NO: 440 - protein, 112 aa, synthetic construct; identical to SEQ ID NO: 392
  REGION 1..112: note = Synthetic

SEQ ID NO: 441 - protein, 116 aa, synthetic construct; identical to SEQ ID NO: 419
  REGION 1..116: note = Synthetic

SEQ ID NO: 442 - protein, 112 aa, synthetic construct; identical to SEQ ID NO: 400
  REGION 1..112: note = Synthetic

SEQ ID NO: 443 - protein, 116 aa, synthetic construct
  REGION 1..116: note = Synthetic
EVQLVQSGAEVKKPGASVKVSCKASGYTFTNYWLGWIKQAPGQGLEWIGDIYPGGDYIVYNEKFKGKATLTADTSISTAYMELSRLRSDDTAVYYCARPNLPKDHWGQGTTVTVSS

SEQ ID NO: 444 - protein, 112 aa, synthetic construct
  REGION 1..112: note = Synthetic
DIVMTQSPLSLPVTPGEPASISCRSSKSLLHSQGITYLYWYLQKPGQSPQLLIYQVSNLASGVPDRFSGSGSGTDFTLKISRVEAEDVGVYYCAQYLELPWTFGGGTKVEIK

SEQ ID NO: 445 - protein, 116 aa, synthetic construct; identical to SEQ ID NO: 443
  REGION 1..116: note = Synthetic

SEQ ID NO: 446 - protein, 112 aa, synthetic construct
  REGION 1..112: note = Synthetic
DIVMTQSPLSLPVTPGEPASISCRSSKSLLHSNAITYLYWYLQKPGQSPQLLIYQVSNLASGVPDRFSGSGSGTDFTLKISRVEAEDVGVYYCGQYLELPWTFGGGTKVEIK

SEQ ID NO: 447 - protein, 116 aa, synthetic construct
  REGION 1..116: note = Synthetic
EVQLVQSGAEVKKPGASVKVSCKASGYLFTNYWLGWIKQAPGQGLEWIGDIYPGGDYIVYNEKFKGKATLTADTSISTAYMELSRLRSDDTAVYYCARPNLPKDHWGQGTTVTVSS

SEQ ID NO: 448 - protein, 112 aa, synthetic construct; identical to SEQ ID NO: 400
  REGION 1..112: note = Synthetic

SEQ ID NO: 449 - protein, 116 aa, synthetic construct; identical to SEQ ID NO: 447
  REGION 1..116: note = Synthetic

SEQ ID NO: 450 - protein, 112 aa, synthetic construct
  REGION 1..112: note = Synthetic
DIVMTQSPLSLPVTPGEPASISCRSSKSLLHSNAITYLYWYLQKPGQSPQLLIYQVSNLATGVPDRFSGSGSGTDFTLKISRVEAEDVGVYYCAQYLELPWTFGGGTKVEIK

SEQ ID NO: 451 - protein, 116 aa, synthetic construct; identical to SEQ ID NO: 447
  REGION 1..116: note = Synthetic

SEQ ID NO: 452 - protein, 112 aa, synthetic construct
  REGION 1..112: note = Synthetic
DIVMTQSPLSLPVTPGEPASISCRSSKSLLHSNAITYLYWYLQKPGQSPQLLIYQVSNLATGVPDRFSGSGSGTDFTLKISRVEAEDVGVYYCGQYLELPWTFGGGTKVEIK

SEQ ID NO: 453 - protein, 10 aa, synthetic construct
  REGION 1..10: note = Synthetic
GYTFENYWLG

SEQ ID NO: 454 - protein, 10 aa, synthetic construct
  REGION 1..10: note = Synthetic
GYMFTNYWLG

SEQ ID NO: 455 - protein, 10 aa, synthetic construct
  REGION 1..10: note = Synthetic
GYTFDNYWLG

SEQ ID NO: 456 - protein, 10 aa, synthetic construct
  REGION 1..10: note = Synthetic
GYTFGNYWLG

SEQ ID NO: 457 - protein, 10 aa, synthetic construct
  REGION 1..10: note = Synthetic
GYTFTNYWLW

SEQ ID NO: 458 - protein, 10 aa, synthetic construct
  REGION 1..10: note = Synthetic
GYLFTNYWLG

SEQ ID NO: 459 - protein, 10 aa, synthetic construct
  REGION 1..10: note = Synthetic
GYTFTNYWLS

SEQ ID NO: 460 - protein, 10 aa, synthetic construct
  REGION 1..10: note = Synthetic
GFTFTNYWLG

SEQ ID NO: 461 - protein, 17 aa, synthetic construct
  REGION 1..17: note = Synthetic
DIYPGGDYIVYNEKFKG

SEQ ID NO: 462 - protein, 17 aa, synthetic construct
  REGION 1..17: note = Synthetic
DIYPGGDIINYNEKFKG

SEQ ID NO: 463 - protein, 17 aa, synthetic construct
  REGION 1..17: note = Synthetic
DIYPGGDVINYNEKFKG

SEQ ID NO: 464 - protein, 17 aa, synthetic construct
  REGION 1..17: note = Synthetic
DIFPGGDYINYNEKFKG

SEQ ID NO: 465 - protein, 17 aa, synthetic construct
  REGION 1..17: note = Synthetic
DIYPGGDLINYNEKFKG

SEQ ID NO: 466 - protein, 17 aa, synthetic construct
  REGION 1..17: note = Synthetic
DIYPGGDHINYNEKFKG

SEQ ID NO: 467 - protein, 17 aa, synthetic construct
  REGION 1..17: note = Synthetic
EIYPGGDYITYNEKFKG

SEQ ID NO: 468 - protein, 7 aa, synthetic construct
  REGION 1..7: note = Synthetic
PNLPKDH

SEQ ID NO: 469 - protein, 7 aa, synthetic construct
  REGION 1..7: note = Synthetic
PDLPGDY

SEQ ID NO: 470 - protein, 7 aa, synthetic construct
  REGION 1..7: note = Synthetic
PGLPKDY

SEQ ID NO: 471 - protein, 7 aa, synthetic construct
  REGION 1..7: note = Synthetic
PNLPKDY

SEQ ID NO: 472 - protein, 7 aa, synthetic construct
  REGION 1..7: note = Synthetic
PNLPRDY

SEQ ID NO: 473 - protein, 7 aa, synthetic construct
  REGION 1..7: note = Synthetic
PGLPRDY

SEQ ID NO: 474 - protein, 7 aa, synthetic construct
  REGION 1..7: note = Synthetic
PGLPQDY

SEQ ID NO: 475 - protein, 7 aa, synthetic construct
  REGION 1..7: note = Synthetic
PDLPKDY

SEQ ID NO: 476 - protein, 7 aa, synthetic construct
  REGION 1..7: note = Synthetic
QVSNLAR

SEQ ID NO: 477 - protein, 7 aa, synthetic construct
  REGION 1..7: note = Synthetic
QKSNLAS

SEQ ID NO: 478 - protein, 7 aa, synthetic construct
  REGION 1..7: note = Synthetic
QVSNLAV

SEQ ID NO: 479 - protein, 7 aa, synthetic construct
  REGION 1..7: note = Synthetic
QVSNLAL

SEQ ID NO: 480 - protein, 7 aa, synthetic construct
  REGION 1..7: note = Synthetic
QVDNLAS

SEQ ID NO: 481 - protein, 7 aa, synthetic construct
  REGION 1..7: note = Synthetic
QVSNLAT

SEQ ID NO: 482 - protein, 7 aa, synthetic construct
  REGION 1..7: note = Synthetic
HVSNLAS

SEQ ID NO: 483 - protein, 7 aa, synthetic construct
  REGION 1..7: note = Synthetic
QVSNRAS

SEQ ID NO: 484 - protein, 9 aa, synthetic construct
  REGION 1..9: note = Synthetic
GQNLELPWT

SEQ ID NO: 485 - protein, 9 aa, synthetic construct
  REGION 1..9: note = Synthetic
AQNLEMPWT

SEQ ID NO: 486 - protein, 9 aa, synthetic construct
  REGION 1..9: note = Synthetic
GQNLEMPWT

SEQ ID NO: 487 - protein, 9 aa, synthetic construct
  REGION 1..9: note = Synthetic
AQYLEEPWT

SEQ ID NO: 488 - protein, 9 aa, synthetic construct
  REGION 1..9: note = Synthetic
AQYLELPWT

SEQ ID NO: 489 - protein, 9 aa, synthetic construct
  REGION 1..9: note = Synthetic
GQYLELPWT

SEQ ID NO: 490 - protein, 16 aa, synthetic construct
  REGION 1..16: note = Synthetic
RSSKSLLHSQGITYLY

SEQ ID NO: 491 - protein, 116 aa, synthetic construct; identical to SEQ ID NO: 443
  REGION 1..116: note = Synthetic

SEQ ID NO: 492 - protein, 112 aa, synthetic construct; identical to SEQ ID NO: 400
  REGION 1..112: note = Synthetic

SEQ ID NO: 493 - protein, 119 aa, synthetic construct
  REGION 1..119: note = Synthetic
EVQLVESGGGLVQPGGSLRLSCAASGFTFSSYDMSWVRQAPGKSLEWVATISDAGGYIYYRDSVKGRFTISRDNAKNSLYLQMNSLRDEDTAVYICAREFGKRYALDYWGQGTTVTVSS

SEQ ID NO: 494 - protein, 107 aa, synthetic construct; identical to SEQ ID NO: 28
  REGION 1..107: note = Synthetic

SEQ ID NO: 495 - protein, 119 aa, synthetic construct; identical to SEQ ID NO: 493
  REGION 1..119: note = Synthetic

SEQ ID NO: 496 - protein, 107 aa, synthetic construct
  REGION 1..107: note = Synthetic
DIQMTQSPSSLSASVGDRVTITCKAKQDVTPAVAWYQQKPGKAPKLLIYSTSSRYTGVPSRFSGSGSGTDFTFTISSLQPEDIATYYCMQHYTTPLTFGQGTKLEIK

SEQ ID NO: 497 - protein, 119 aa, synthetic construct
  REGION 1..119: note = Synthetic
EVQLVESGGGLVQPGGSLRLSCAASGFTFSSYDMSWVRQAPGKSLEWVATISDAGGYIYYRDSVKGRFTISRDNAKNSLYLQMNSLRDEDTAVYICAREFGKRYALDSWGQGTTVTVSS

SEQ ID NO: 498 - protein, 107 aa, synthetic construct
  REGION 1..107: note = Synthetic
DIQMTQSPSSLSASVGDRVTITCKASQDVWPAVAWYQQKPGKAPKLLIYSTSSRYTGVPSRFSGSGSGTDFTFTISSLQPEDIATYYCQQHSTTPLTFGQGTKLEIK

SEQ ID NO: 499 - protein, 119 aa, synthetic construct
  REGION 1..119: note = Synthetic
EVQLVESGGGLVQPGGSLRLSCAASGFTFSSYDMSWVRQAPGKSLEWVATISDAGGYIYYRDSVKGRFTISRDNAKNSLYLQMNSLRDEDTAVYICAREIFNRYALDYWGQGTTVTVSS

SEQ ID NO: 500 - protein, 107 aa, synthetic construct; identical to SEQ ID NO: 28
  REGION 1..107: note = Synthetic

SEQ ID NO: 501 - protein, 119 aa, synthetic construct
  REGION 1..119: note = Synthetic
EVQLVESGGGLVQPGGSLRLSCAASGFTFSSYDMSWVRQAPGKSLEWVATISDAGGYIYYRDSVKGRFTISRDNAKNSLYLQMNSLRDEDTAVYICARELPWRYALDYWGQGTTVTVSS

SEQ ID NO: 502 - protein, 107 aa, synthetic construct; identical to SEQ ID NO: 28
  REGION 1..107: note = Synthetic

SEQ ID NO: 503 - protein, 119 aa, synthetic construct
  REGION 1..119: note = Synthetic
EVQLVESGGGLVQPGGSLRLSCAASGFTFSSYDMSWVRQAPGKSLEWVATISDAGGYIYYRDSVKGRFTISRDNAKNSLYLQMNSLRDEDTAVYICARELHFRYALDYWGQGTTVTVSS

SEQ ID NO: 504 - protein, 107 aa, synthetic construct; identical to SEQ ID NO: 28
  REGION 1..107: note = Synthetic

SEQ ID NO: 505 - protein, 119 aa, synthetic construct
  REGION 1..119: note = Synthetic
EVQLVESGGGLVQPGGSLRLSCAASGFTFSSYDMSWVRQAPGKSLEWVATISDAGGYIYYRDSVKGRFTISRDNAKNSLYLQMNSLRDEDTAVYICARELYFRYALDYWGQGTTVTVSS

SEQ ID NO: 506 - protein, 107 aa, synthetic construct; identical to SEQ ID NO: 28
  REGION 1..107: note = Synthetic

SEQ ID NO: 507 - protein, 119 aa, synthetic construct
  REGION 1..119: note = Synthetic
EVQLVESGGGLVQPGGSLRLSCAASGFTFSSYDMSWVRQAPGKSLEWVATISDAGGYIYYRDSVKGRFTISRDNAKNSLYLQMNSLRDEDTAVYICARELLHRYALDYWGQGTTVTVSS

SEQ ID NO: 508 - protein, 107 aa, synthetic construct; identical to SEQ ID NO: 28
  REGION 1..107: note = Synthetic

SEQ ID NO: 509 - protein, 119 aa, synthetic construct
  REGION 1..119: note = Synthetic
EVQLVESGGGLVQPGGSLRLSCAASGFTFSSYDMSWVRQAPGKSLEWVATISDAGGYIYYRDSVKGRFTISRDNAKNSLYLQMNSLRDEDTAVYICARELRGRYALDYWGQGTTVTVSS

SEQ ID NO: 510 - protein, 107 aa, synthetic construct; identical to SEQ ID NO: 28
  REGION 1..107: note = Synthetic

SEQ ID NO: 511 - protein, 119 aa, synthetic construct; identical to SEQ ID NO: 493
  REGION 1..119: note = Synthetic

SEQ ID NO: 512 - protein, 107 aa, synthetic construct
  REGION 1..107: note = Synthetic
DIQMTQSPSSLSASVGDRVTITCKASQDVTPAVAWYQQKPGKAPKLLIYSTSSRYTGVPSRFSGSGSGTDFTFTISSLQPEDIATYYCQQHSDAPLTFGQGTKLEIK

SEQ ID NO: 513 - protein, 10 aa, synthetic construct
  REGION 1..10: note = Synthetic
EFGKRYALDS

SEQ ID NO: 514 - protein, 10 aa, synthetic construct
  REGION 1..10: note = Synthetic
EIFNRYALDY

SEQ ID NO: 515 - protein, 10 aa, synthetic construct
  REGION 1..10: note = Synthetic
ELPWRYALDY

SEQ ID NO: 516 - protein, 10 aa, synthetic construct
  REGION 1..10: note = Synthetic
ELHFRYALDY

SEQ ID NO: 517 - protein, 10 aa, synthetic construct
  REGION 1..10: note = Synthetic
ELYFRYALDY

SEQ ID NO: 518 - protein, 10 aa, synthetic construct
  REGION 1..10: note = Synthetic
ELLHRYALDY

SEQ ID NO: 519 - protein, 10 aa, synthetic construct
  REGION 1..10: note = Synthetic
ELRGRYALDY

SEQ ID NO: 520 - protein, 11 aa, synthetic construct
  REGION 1..11: note = Synthetic
KAKQDVTPAVA

SEQ ID NO: 521 - protein, 11 aa, synthetic construct
  REGION 1..11: note = Synthetic
KASQDVWPAVA

SEQ ID NO: 522 - protein, 9 aa, synthetic construct
  REGION 1..9: note = Synthetic
MQHYTTPLT

SEQ ID NO: 523 - protein, 9 aa, synthetic construct
  REGION 1..9: note = Synthetic
QQHSTTPLT

SEQ ID NO: 524 - protein, 9 aa, synthetic construct
  REGION 1..9: note = Synthetic
QQHSDAPLT

SEQ ID NO: 525 - protein, 17 aa, synthetic construct
  REGION 1..17: note = Synthetic
TISDAGGYIYYSDSVKG

SEQ ID NO: 526 - protein, 17 aa, synthetic construct
  REGION 1..17: note = Synthetic
TISDAGGYIYYRDSVKG

SEQ ID NO: 527 - protein, 17 aa, synthetic construct
  REGION 1..17: note = Synthetic
TISDGGGYIYYRDSVKG

SEQ ID NO: 528 - protein, 449 aa, synthetic construct
  REGION 1..449: note = Synthetic
EVQLVESGGGLVQPGGSLRLSCAASGFTFSSYDMSWVRQAPGKSLEWVATISDAGGYIYYSDSVKGRFTISRDNAKNSLYLQMNSLRDEDTAVYICAREFGKRYALDYWGQGTTVTVSSASTKGPSVFPLAPSSKSTSGGTAALGCLVKDYFPEPVTVSWNSGALTSGVHTFPAVLQSSGLYSLSSVVTVPSSSLGTQTYICNVNHKPSNTKVDKKVEPKSCDKTHTCPPCPAPELLGGPSVFLFPPKPKDTLMISRTPEVTCVVVDVSHEDPEVKFNWYVDGVEVHNAKTKPREEQYASTYRVVSVLTVLHQDWLNGKEYKCKVSNKALPAPIEKTISKAKGQPREPQVYTLPPSREEMTKNQVSLTCLVKGFYPSDIAVEWESNGQPENNYKTTPPVLDSDGSFFLYSKLTVDKSRWQQGNVFSCSVMHEALHNHYTQKSLSLSPGK

SEQ ID NO: 529 - protein, 18 aa, synthetic construct
  REGION 1..18: note = Synthetic
GSGSGSGSGSGSGSGSGS

SEQ ID NO: 530 - protein, 113 aa, synthetic construct
  REGION 1..113: note = Synthetic
DIVMTQSPLSLPVTPGEPASISCRSSKSLLHSNGITYLYWYLQKPGQSPQLLIYQVSNLASGVPDRFSGSGSGTDFTLKISRVEAEDVGVYYCAQNLELPWTFGCGTKVEIKR

SEQ ID NO: 531 - protein, 20 aa, synthetic construct
  REGION 1..20: note = Synthetic
GGGGSGGGGSGGGGSGGGGS

SEQ ID NO: 532 - protein, 116 aa, synthetic construct
  REGION 1..116: note = Synthetic
EVQLVQSGAEVKKPGASVKVSCKASGYTFTNYWLGWIKQAPGQCLEWIGDIYPGGDYINYNEKFKGKATLTADTSISTAYMELSRLRSDDTAVYYCARPNLPGDYWGQGTTVTVSS

SEQ ID NO: 533 - DNA, 2151 bp, synthetic construct
  misc_feature 1..2151: note = Synthetic
  source 1..2151: mol_type = other DNA
gaggtgcagctggtggagagcggaggaggactggtgcaacccggaggcagcctgagactgagctgcgctgccagcggcttcaccttcagcagctacgacatgagctgggtgagacaggcccctggcaaaagcctggagtgggtggccaccatctccgatgcgggcggctacatctattactccgacagcgtgaagggcaggttcaccatcagcagggacaacgccaagaacagcctgtacctgcagatgaacagcctgagggatgaggacaccgccgtgtacatctgcgccagggagttcggcaaaaggtacgccctggactactggggccagggcacaaccgtgaccgtgagcagcgctagcaccaagggcccctctgtgttccctctggccccttcctctaaatccacctctggcggaaccgctgctctgggctgtctggtcaaggactacttccctgagcccgtgaccgtgtcttggaattctggcgctctgaccagcggagtgcacacctttccagctgtgctgcagtcctccggcctgtactctctgtcctctgtcgtgacagtgccttccagctctctgggcacccagacctacatctgcaacgtgaaccacaagccctccaacaccaaggtggacaagaaggtggaacccaagtcctgcgacaagacccacacctgtcctccatgtcctgctccagaactgctgggcggaccctccgtgttcctgttccctccaaagcctaaggacaccctgatgatctcccggacccctgaagtgacctgcgtggtggtggatgtgtcccacgaggatcccgaagtgaagttcaattggtacgtggacggcgtggaagtgcacaacgccaagaccaagcctagagaggaacagtacgcctccacctaccgggtggtgtccgtgctgaccgttctgcaccaggattggctgaacggcaaagagtacaagtgcaaggtgtccaacaaggccctgcctgcccctatcgaaaagaccatctctaaggccaagggccagccccgggaacctcaagtgtacaccttgcctcccagccgggaagagatgaccaagaaccaggtgtccctgacctgcctggttaagggcttctacccctccgatatcgccgtggaatgggagtctaatggccagcctgagaacaactacaagaccacacctcctgtgctggactccgacggctcattcttcctgtactccaagctgaccgtggacaagtccagatggcagcagggcaacgtgttctcctgctccgtgatgcacgaggccctgcacaatcactacacccagaagtccctgtctctgtcccctggcaaaggctccggatctggttctggatccggaagcggttctggcagcggctctggatctgacatcgtgatgacccagtctccactgagcctgcctgtgacacctggcgagcctgcttccatctcctgccggtcctctaagtccctgctgcactctaacggcatcacctacctgtactggtatctgcagaagcccggccagtctcctcagctgctgatctaccaggtgtccaacctggcttctggcgtgcccgatagattctccggtagcggatctggaaccgacttcaccctgaagatctccagagtggaagccgaggacgtgggcgtgtactactgtgcccagaacctggaactgccctggacctttggctgtggcaccaaggtggaaatcaagagaggcggcggaggatctggcggaggtggaagcggaggcggaggaagcggtggcggcggatctgaagttcagttggttcagtctggcgccgaagtgaagaaacctggcgcctctgtgaaggtgtcctgcaaggcttccggctacacctttaccaactactggctcggctggatcaagcaggcccctggacagtgtctggaatggatcggcgacatctaccctggcggcgactacatcaactacaacgagaagttcaagggcaaagctaccctgaccgccgacacctctatctccaccgcctacatggaactgtcccggctgagatctgacgacaccgccgtgtactattgcgccagacctaacctgcctggcgactattggggccagggcacaacagtgaccgtgtcctcttaa

SEQ ID NO: 534 - protein, 214 aa, synthetic construct
  REGION 1..214: note = Synthetic
DIQMTQSPSSLSASVGDRVTITCKASQDVTPAVAWYQQKPGKAPKLLIYSTSSRYTGVPSRFSGSGSGTDFTFTISSLQPEDIATYYCQQHYTTPLTFGQGTKLEIKRTVAAPSVFIFPPSDEQLKSGTASVVCLLNNFYPREAKVQWKVDNALQSGNSQESVTEQDSKDSTYSLSSTLTLSKADYEKHKVYACEVTHQGLSSPVTKSFNRGEC

SEQ ID NO: 535 - DNA, 645 bp, synthetic construct
  misc_feature 1..645: note = Synthetic
  source 1..645: mol_type = other DNA
gacatccagatgacccagagccctagcagcctgagcgctagcgtgggcgacagggtgaccatcacctgcaaggccagccaggatgtgacccctgccgtggcctggtaccagcagaagcccggcaaggcccccaagctgctgatctacagcaccagcagcaggtacaccggcgtgcccagcaggtttagcggaagcggcagcggcaccgacttcaccttcaccatcagcagcctgcagcccgaggacatcgccacctactactgccagcagcactacaccacccctctgaccttcggccagggcaccaagctggagatcaagagaaccgtggccgctccctccgtgttcatcttcccaccatctgacgagcagctgaagtccggcaccgcttctgtcgtgtgcctgctgaacaacttctaccctcgggaagccaaggtgcagtggaaggtggacaatgccctgcagtccggcaactcccaagagtctgtgaccgagcaggactccaaggacagcacctactccctgtcctctaccctgaccctgtccaaggccgactacgagaagcacaaggtgtacgcctgcgaagtgacccaccagggactgtctagccccgtgaccaagtccttcaacagaggcgagtgctga

SEQ ID NO: 536 - protein, 113 aa, synthetic construct
  REGION 1..113: note = Synthetic
DIVMTQSPLSLPVTPGEPASISCRSSKSLLHSQGITYLYWYLQKPGQSPQLLIYQVSNLASGVPDRFSGSGSGTDFTLKISRVEAEDVGVYYCAQYLELPWTFGCGTKVEIKR

SEQ ID NO: 537 - protein, 116 aa, synthetic construct
  REGION 1..116: note = Synthetic
EVQLVQSGAEVKKPGASVKVSCKASGYTFTNYWLGWIKQAPGQCLEWIGDIYPGGDYIVYNEKFKGKATLTADTSISTAYMELSRLRSDDTAVYYCARPNLPKDHWGQGTTVTVSS

SEQ ID NO: 538 - DNA, 2151 bp, synthetic construct
  misc_feature 1..2151: note = Synthetic
  source 1..2151: mol_type = other DNA
gaggtgcagctggtggagagcggaggaggactggtgcaacccggaggcagcctgagactgagctgcgctgccagcggcttcaccttcagcagctacgacatgagctgggtgagacaggcccctggcaaaagcctggagtgggtggccaccatctccgatgcgggcggctacatctattactccgacagcgtgaagggcaggttcaccatcagcagggacaacgccaagaacagcctgtacctgcagatgaacagcctgagggatgaggacaccgccgtgtacatctgcgccagggagttcggcaaaaggtacgccctggactactggggccagggcacaaccgtgaccgtgagcagcgctagcaccaagggcccctctgtgttccctctggccccttcctctaaatccacctctggcggaaccgctgctctgggctgtctggtcaaggactacttccctgagcccgtgaccgtgtcttggaattctggcgctctgaccagcggagtgcacacctttccagctgtgctgcagtcctccggcctgtactctctgtcctctgtcgtgacagtgccttccagctctctgggcacccagacctacatctgcaacgtgaaccacaagccctccaacaccaaggtggacaagaaggtggaacccaagtcctgcgacaagacccacacctgtcctccatgtcctgctccagaactgctgggcggaccctccgtgttcctgttccctccaaagcctaaggacaccctgatgatctcccggacccctgaagtgacctgcgtggtggtggatgtgtcccacgaggatcccgaagtgaagttcaattggtacgtggacggcgtggaagtgcacaacgccaagaccaagcctagagaggaacagtacgcctccacctaccgggtggtgtccgtgctgaccgttctgcaccaggattggctgaacggcaaagagtacaagtgcaaggtgtccaacaaggccctgcctgcccctatcgaaaagaccatctctaaggccaagggccagccccgggaacctcaagtgtacaccttgcctcccagccgggaagagatgaccaagaaccaggtgtccctgacctgcctggttaagggcttctacccctccgatatcgccgtggaatgggagtctaacggccagcccgagaacaactacaagaccacccctcctgtgctggactccgacggctcattcttcctgtactccaagctgaccgtggacaagtctcggtggcagcagggcaacgtgttctcctgctctgtgatgcacgaggccctgcacaaccactacacccagaagtccctgtccctgtctcccggcaaaggctccggatctggttctggatccggaagcggttctggcagcggctctggatctgacattgtgatgacccagagccccctgagcctccccgtgacccctggagaacccgccagcataagctgcagatcctccaaaagcctgctgcactcccagggaataacctacctgtattggtacctgcagaaacccggccaatccccccaactcctgatataccaagtgtccaacctggcctccggcgtgcccgacagattctccggctccggcagcggtaccgacttcaccctcaaaatctccagagtggaagcagaagacgtcggcgtgtactactgcgcccagtacctggaactgccctggaccttcggctgtggcaccaaggtggaaatcaagagaggcggcggaggaagcggaggcggcggttctggtggtggcggtagcggaggtggtggatctgaggtgcagctggtgcagagcggagcagaggtgaagaagccaggggccagcgtgaaggtgagctgtaaggctagtgggtacacatttacaaactattggctgggatggattaagcaggccccaggccaatgcctggagtggataggagacatataccccggaggagactatatcgtgtacaacgagaagttcaagggcaaggccacactcaccgctgatacaagcatcagcaccgcctacatggagctgagccgactgagaagcgacgacacagcagtgtattactgcgccagacccaacctgcccaaggaccactggggacaaggcaccaccgtgaccgtgagcagctga

SEQ ID NO: 539 - protein, 449 aa, synthetic construct
  REGION 1..449: note = Synthetic
EVQLVESGGGLVQPGGSLRLSCAASGFTFSSYDMSWVRQAPGKSLEWVATISDAGGYIYYRDSVKGRFTISRDNAKNSLYLQMNSLRDEDTAVYICARELPWRYALDYWGQGTTVTVSSASTKGPSVFPLAPSSKSTSGGTAALGCLVKDYFPEPVTVSWNSGALTSGVHTFPAVLQSSGLYSLSSVVTVPSSSLGTQTYICNVNHKPSNTKVDKKVEPKSCDKTHTCPPCPAPELLGGPSVFLFPPKPKDTLMISRTPEVTCVVVDVSHEDPEVKFNWYVDGVEVHNAKTKPREEQYASTYRVVSVLTVLHQDWLNGKEYKCKVSNKALPAPIEKTISKAKGQPREPQVYTLPPSREEMTKNQVSLTCLVKGFYPSDIAVEWESNGQPENNYKTTPPVLDSDGSFFLYSKLTVDKSRWQQGNVFSCSVMHEALHNHYTQKSLSLSPGK

SEQ ID NO: 540 - DNA, 2151 bp, synthetic construct
  misc_feature 1..2151: note = Synthetic
  source 1..2151: mol_type = other DNA
gaagtgcagctggttgaatctggcggcggattggttcagcctggcggatctctgagactgtcttgtgccgcctccggcttcaccttctccagctacgatatgtcctgggtccgacaggcccctggcaagtctttggaatgggtcgccaccatctctgacgctggcggctacatctactaccgggactctgtgaagggcagattcaccatcagccgggacaacgccaagaactccctgtacctgcagatgaacagcctgcgcgacgaggataccgccgtgtacatctgtgctagagagctgccttggagatacgccctggattattggggccagggcaccacagtgaccgtgtcctctgcttctaccaagggacccagcgtgttccctctggctccttccagcaagtctacctctggcggaacagctgctctgggctgcctggtcaaggactactttcctgagcctgtgacagtgtcctggaactctggcgctctgacatctggcgtgcacacctttccagcagtgctgcagtcctccggcctgtactctctgtcctctgtcgtgaccgtgccttccagctctctgggcacccagacctacatctgcaacgtgaaccacaagccctccaacaccaaggtggacaagaaggtggaacccaagtcctgcgacaagacccacacctgtcctccatgtcctgctccagaactgctgggcggaccctccgtgttcctgttccctccaaagcctaaggacaccctgatgatctcccggacccctgaagtgacctgcgtggtggtggatgtgtcccacgaggatcccgaagtgaagttcaattggtacgtggacggcgtggaagtgcacaacgccaagaccaagcctagagaggaacagtacgcctccacctaccgggtggtgtccgtgctgaccgttctgcaccaggattggctgaacggcaaagagtacaagtgcaaggtgtccaacaaggccctgcctgcccctatcgaaaagaccatctctaaggccaagggccagccccgggaacctcaagtgtacaccttgcctcccagccgggaagagatgaccaagaaccaggtgtccctgacctgcctggttaagggcttctacccctccgatatcgccgtggaatgggagtctaatggccagcctgagaacaactacaagaccacacctcctgtgctggactccgacggctcattcttcctgtactccaagctgaccgtggacaagtccagatggcagcagggcaacgtgttctcctgctccgtgatgcacgaggccctgcacaatcactacacccagaagtccctgtctctgtcccctggcaaaggctccggatctggttctggatccggaagcggttctggcagcggctctggatctgacatcgtgatgacccagtctccactgagcctgcctgtgacacctggcgagcctgcttccatctcctgccggtcctctaagtccctgctgcactctaacggcatcacctacctgtactggtatctgcagaagcccggccagtctcctcagctgctgatctaccaggtgtccaacctggcttctggcgtgcccgatagattctccggtagcggatctggaaccgacttcaccctgaagatctccagagtggaagccgaggacgtgggcgtgtactactgtgcccagaacctggaactgccctggacctttggctgtggcaccaaggtggaaatcaagagaggcggcggaggatctggcggaggtggaagcggaggcggaggaagcggtggcggcggatctgaagttcagttggttcagtctggcgccgaagtgaagaaacctggcgcctctgtgaaggtgtcctgcaaggcttccggctacacctttaccaactactggctcggctggatcaagcaggcccctggacagtgtctggaatggatcggcgacatctaccctggcggcgactacatcaactacaacgagaagttcaagggcaaagctaccctgaccgccgacacctctatctccaccgcctacatggaactgtcccggctgagatctgacgacaccgccgtgtactattgcgccagacctaacctgcctggcgactattggggccagggcacaacagtgaccgtgtcctcttaa

SEQ ID NO: 541 - DNA, 2151 bp, synthetic construct
  misc_feature 1..2151: note = Synthetic
  source 1..2151: mol_type = other DNA
gaagtgcagctggttgaatctggcggcggattggttcagcctggcggatctctgagactgtcttgtgccgcctccggcttcaccttctccagctacgatatgtcctgggtccgacaggcccctggcaagtctttggaatgggtcgccaccatctctgacgctggcggctacatctactaccgggactctgtgaagggcagattcaccatcagccgggacaacgccaagaactccctgtacctgcagatgaacagcctgcgcgacgaggataccgccgtgtacatctgtgctagagagctgccttggagatacgccctggattattggggccagggcaccacagtgaccgtgtcctctgcttctaccaagggacccagcgtgttccctctggctccttccagcaagtctacctctggcggaacagctgctctgggctgcctggtcaaggactactttcctgagcctgtgacagtgtcctggaactctggcgctctgacatctggcgtgcacacctttccagcagtgctgcagtcctccggcctgtactctctgtcctctgtcgtgaccgtgccttccagctctctgggcacccagacctacatctgcaacgtgaaccacaagccctccaacaccaaggtggacaagaaggtggaacccaagtcctgcgacaagacccacacctgtcctccatgtcctgctccagaactgctgggcggaccctccgtgttcctgttccctccaaagcctaaggacaccctgatgatctcccggacccctgaagtgacctgcgtggtggtggatgtgtcccacgaggatcccgaagtgaagttcaattggtacgtggacggcgtggaagtgcacaacgccaagaccaagcctagagaggaacagtacgcctccacctaccgggtggtgtccgtgctgaccgttctgcaccaggattggctgaacggcaaagagtacaagtgcaaggtgtccaacaaggccctgcctgcccctatcgaaaagaccatctctaaggccaagggccagccccgggaacctcaagtgtacaccttgcctcccagccgggaagagatgaccaagaaccaggtgtccctgacctgcctggttaagggcttctacccctccgatatcgccgtggaatgggagtctaacggccagcccgagaacaactacaagaccacccctcctgtgctggactccgacggctcattcttcctgtactccaagctgaccgtggacaagtctcggtggcagcagggcaacgtgttctcctgctctgtgatgcacgaggccctgcacaaccactacacccagaagtccctgtccctgtctcccggcaaaggctccggatctggttctggatccggaagcggttctggcagcggctctggatctgacattgtgatgacccagagccccctgagcctccccgtgacccctggagaacccgccagcataagctgcagatcctccaaaagcctgctgcactcccagggaataacctacctgtattggtacctgcagaaacccggccaatccccccaactcctgatataccaagtgtccaacctggcctccggcgtgcccgacagattctccggctccggcagcggtaccgacttcaccctcaaaatctccagagtggaagcagaagacgtcggcgtgtactactgcgcccagtacctggaactgccctggaccttcggctgtggcaccaaggtggaaatcaagagaggcggcggaggaagcggaggcggcggttctggtggtggcggtagcggaggtggtggatctgaggtgcagctggtgcagagcggagcagaggtgaagaagccaggggccagcgtgaaggtgagctgtaaggctagtgggtacacatttacaaactattggctgggatggattaagcaggccccaggccaatgcctggagtggataggagacatataccccggaggagactatatcgtgtacaacgagaagttcaagggcaaggccacactcaccgctgatacaagcatcagcaccgcctacatggagctgagccgactgagaagcgacgacacagcagtgtattactgcgccagacccaacctgcccaaggaccactggggacaaggcaccaccgtgaccgtgagcagctga

SEQ ID NO: 542 - protein, 443 aa, synthetic construct
  REGION 1..443: note = Synthetic
EVQLVQSGAEVKKPGASVKVSCKASGYTFTNYWLGWIKQAPGQGLEWIGDIYPGGDYINYNEKFKGKATLTADTSISTAYMELSRLRSDDTAVYYCARPNLPGDYWGQGTTVTVSSASTKGPSVFPLAPCSRSTSESTAALGCLVKDYFPEPVTVSWNSGALTSGVHTFPAVLQSSGLYSLSSVVTVPSSSLGTKTYTCNVDHKPSNTKVDKRVESKYGPPCPPCPAPEFLGGPSVFLFPPKPKDTLMISRTPEVTCVVVDVSQEDPEVQFNWYVDGVEVHNAKTKPREEQFNSTYRVVSVLTVLHQDWLNGKEYKCKVSNKGLPSSIEKTISKAKGQPREPQVYTLPPSQEEMTKNQVSLTCLVKGFYPSDIAVEWESNGQPENNYKTTPPVLDSDGSFFLYSRLTVDKSRWQEGNVFSCSVMHEALHNHYTQKSLSLSLGK

SEQ ID NO: 543 - protein, 15 aa, synthetic construct
  REGION 1..15: note = Synthetic
GGGGSGGGGSGGGGS

SEQ ID NO: 544 - protein, 108 aa, synthetic construct
  REGION 1..108: note = Synthetic
DIQMTQSPSSLSASVGDRVTITCKASQDVTPAVAWYQQKPGKAPKLLIYSTSSRYTGVPSRFSGSGSGTDFTFTISSLQPEDIATYYCQQHYTTPLTFGCGTKLEIKR

SEQ ID NO: 545 - protein, 119 aa, synthetic construct
  REGION 1..119: note = Synthetic
EVQLVESGGGLVQPGGSLRLSCAASGFTFSSYDMSWVRQAPGKCLEWVATISDAGGYIYYSDSVKGRFTISRDNAKNSLYLQMNSLRDEDTAVYICAREFGKRYALDYWGQGTTVTVSS

SEQ ID NO: 546 - DNA, 2118 bp, synthetic construct
  misc_feature 1..2118: note = Synthetic
  source 1..2118: mol_type = other DNA
gaggtgcagctggtgcagagcggagcagaggtgaagaagccaggggccagcgtgaaggtgagctgtaaggctagtgggtacacatttacaaactattggctgggatggattaagcaggccccaggccaaggactggagtggataggagacatataccccggaggagactatatcaattacaacgagaagttcaagggcaaggccacactcaccgctgatacaagcatcagcaccgcctacatggagctgagccgactgagaagcgacgacacagcagtgtattactgcgccagacccaacctgcccggcgactactggggacaaggcaccaccgtgaccgtgtcttccgctagcaccaagggcccctccgtgttccctctggccccatgctcccggtccacctccgagtccaccgccgctctgggctgtctggtgaaggactacttccctgagcccgtgaccgtgagctggaactctggcgccctgacctccggcgtgcacaccttccctgccgtgctgcagtcctccggcctgtactccctgtcctccgtggtgaccgtgccttcctcctccctgggcaccaagacctacacctgcaacgtggaccacaagccttccaacaccaaggtggacaagcgggtggagtccaagtacggccctccttgccctccctgccctgcccctgagttcctgggcggaccctccgtgttcctgttccctcctaagcctaaggacaccctgatgatctcccggacccctgaggtgacctgcgtggtggtggacgtgtcccaggaagatcctgaggtccagttcaattggtacgtggatggcgtggaggtgcacaacgccaagaccaagcctcgggaggaacagttcaactccacctaccgggtggtgtctgtgctgaccgtgctgcaccaggactggctgaacggcaaggaatacaagtgcaaggtcagcaacaagggcctgccctcctccatcgagaaaaccatctccaaggccaagggccagcctcgcgagcctcaggtgtacaccctgcctcctagccaggaagagatgaccaagaatcaggtgtccctgacatgcctggtgaagggcttctacccttccgatatcgccgtggagtgggagagcaacggccagccagagaacaactacaagaccacccctcctgtgctggactccgacggctccttcttcctgtactccaggctgaccgtggacaagtcccggtggcaggaaggcaacgtcttttcctgctccgtgatgcacgaggccctgcacaaccactacacccagaagtccctgtccctgtctctgggcaagggtggaggtgggtctgggggtggcgggtcaggtggaggaggttcagacatccagatgacccagagccctagcagcctgagcgctagcgtgggcgacagggtgaccatcacctgcaaggccagccaggatgtgacccctgccgtggcctggtaccagcagaagcccggcaaggcccccaagctgctgatctacagcaccagcagcaggtacaccggcgtgcccagcaggtttagcggaagcggcagcggcaccgacttcaccttcaccatcagcagcctgcagcccgaggacatcgccacctactactgccagcagcactacaccacccctctgaccttcggctgtggcaccaagctggagatcaagagaggtggaggcggctcaggggggggtggatcagggggaggaggatcagggggaggcggtagtgaggtgcagctggtggagagcggaggaggactggtgcaacccggaggcagcctgagactgagctgcgctgccagcggcttcaccttcagcagctacgacatgagctgggtgagacaggcccctggcaaatgtctggagtgggtggccaccatctccgatgcgggcggctacatctattactccgacagcgtgaagggcaggttcaccatcagcagggacaacgccaagaacagcctgtacctgcagatgaacagcctgagggatgaggacaccgccgtgtacatctgcgccagggagttcggcaaaaggtacgccctggactactggggccagggcacaaccgtgaccgtgagcagctga

SEQ ID NO: 547 - protein, 219 aa, synthetic construct
  REGION 1..219: note = Synthetic
DIVMTQSPLSLPVTPGEPASISCRSSKSLLHSNGITYLYWYLQKPGQSPQLLIYQVSNLASGVPDRFSGSGSGTDFTLKISRVEAEDVGVYYCAQNLELPWTFGGGTKVEIKRTVAAPSVFIFPPSDEQLKSGTASVVCLLNNFYPREAKVQWKVDNALQSGNSQESVTEQDSKDSTYSLSSTLTLSKADYEKHKVYACEVTHQGLSSPVTKSFNRGEC

SEQ ID NO: 548 - DNA, 660 bp, synthetic construct
  misc_feature 1..660: note = Synthetic
  source 1..660: mol_type = other DNA
gacattgtgatgacccagagccccctgagcctccccgtgacccctggagaacccgccagcataagctgcagatcctccaaaagcctgctgcactccaacggaataacctacctgtattggtacctgcagaaacccggccaatccccccaactcctgatataccaagtgtccaacctggcctccggcgtgcccgacagattctccggctccggcagcggtaccgacttcaccctcaaaatctccagagtggaagcagaagacgtcggcgtgtactactgcgcccagaatctggaactgccctggaccttcggcggcggcaccaaggtggaaatcaagagaaccgtggccgctccctccgtgttcatcttcccaccatctgacgagcagctgaagtccggcaccgcttctgtcgtgtgcctgctgaacaacttctaccctcgggaagccaaggtgcagtggaaggtggacaatgccctgcagtccggcaactcccaagagtctgtgaccgagcaggactccaaggacagcacctactccctgtcctctaccctgaccctgtccaaggccgactacgagaagcacaaggtgtacgcctgcgaagtgacccaccagggactgtctagccccgtgaccaagtccttcaacagaggcgagtgctga

SEQ ID NO: 549 - protein, 119 aa, synthetic construct
  REGION 1..119: note = Synthetic
EVQLVESGGGLVQPGGSLRLSCAASGFTFSSYDMSWVRQAPGKCLEWVATISDAGGYIYYRDSVKGRFTISRDNAKNSLYLQMNSLRDEDTAVYICARELPWRYALDYWGQGTTVTVSS

SEQ ID NO: 550 - DNA, 2118 bp, synthetic construct
  misc_feature 1..2118: note = Synthetic
  source 1..2118: mol_type = other DNA
gaggtgcagctggtgcagagcggagcagaggtgaagaagccaggggccagcgtgaaggtgagctgtaaggctagtgggtacacatttacaaactattggctgggatggattaagcaggccccaggccaaggactggagtggataggagacatataccccggaggagactatatcaattacaacgagaagttcaagggcaaggccacactcaccgctgatacaagcatcagcaccgcctacatggagctgagccgactgagaagcgacgacacagcagtgtattactgcgccagacccaacctgcccggcgactactggggacaaggcaccaccgtgaccgtgtcttccgctagcaccaagggcccctccgtgttccctctggccccatgctcccggtccacctccgagtccaccgccgctctgggctgtctggtgaaggactacttccctgagcccgtgaccgtgagctggaactctggcgccctgacctccggcgtgcacaccttccctgccgtgctgcagtcctccggcctgtactccctgtcctccgtggtgaccgtgccttcctcctccctgggcaccaagacctacacctgcaacgtggaccacaagccttccaacaccaaggtggacaagcgggtggagtccaagtacggccctccttgccctccctgccctgcccctgagttcctgggcggaccctccgtgttcctgttccctcctaagcctaaggacaccctgatgatctcccggacccctgaggtgacctgcgtggtggtggacgtgtcccaggaagatcctgaggtccagttcaattggtacgtggatggcgtggaggtgcacaacgccaagaccaagcctcgggaggaacagttcaactccacctaccgggtggtgtctgtgctgaccgtgctgcaccaggactggctgaacggcaaggaatacaagtgcaaggtcagcaacaagggcctgccctcctccatcgagaaaaccatctccaaggccaagggccagcctcgcgagcctcaggtgtacaccctgcctcctagccaggaagagatgaccaagaatcaggtgtccctgacatgcctggtgaagggcttctacccttccgatatcgccgtggaatgggagagcaatggccagcctgagaacaactacaagacaacccctcctgtgctggactccgacggctccttctttctgtactctcgcctgaccgtggacaagtccagatggcaagagggcaacgtgttctcctgctccgtgatgcacgaggccctgcacaatcactacacccagaagtccctgtctctgtccctcggaaaaggcggcggaggatctggcggaggcggtagcggtggtggcggatctgatattcagatgacccagtctccttccagcctgtccgcttctgtgggcgacagagtgaccatcacatgcaaggccagccaggatgtgacccctgctgtggcttggtatcagcagaagcctggcaaggcccctaagctgctgatctactccacctcctccagatacacaggcgtgccctccagattctccggctctggctctggcaccgactttacctttacaatctccagcctgcagcctgaggacattgccacctactactgccagcagcactacaccacacctctgacctttggctgcggcaccaagctggaaatcaagagaggtggcggaggaagcggaggcggcggttcaggtggcggtggttcaggcggtggtggatctgaagttcagctggtggaatctggcggcggattggttcaaccaggcggctctctgagactgtcttgtgccgcttccggcttcaccttctccagctacgacatgtcctgggtccgacaggcccctggaaagtgtctggaatgggtcgccaccatctctgacgctggcggctacatctactaccgggactctgtgaagggcagattcaccatcagccgggacaatgccaagaactccctgtacctgcagatgaacagtctgcgcgacgaggacaccgccgtgtacatctgtgctagagagctgccttggcgctacgccctggattattggggccagggcacaacagtgacagtgtcctcttga

SEQ ID NO: 551 - protein, 443 aa, synthetic construct
  REGION 1..443: note = Synthetic
EVQLVQSGAEVKKPGASVKVSCKASGYTFTNYWLGWIKQAPGQGLEWIGDIYPGGDYIVYNEKFKGKATLTADTSISTAYMELSRLRSDDTAVYYCARPNLPKDHWGQGTTVTVSSASTKGPSVFPLAPCSRSTSESTAALGCLVKDYFPEPVTVSWNSGALTSGVHTFPAVLQSSGLYSLSSVVTVPSSSLGTKTYTCNVDHKPSNTKVDKRVESKYGPPCPPCPAPEFLGGPSVFLFPPKPKDTLMISRTPEVTCVVVDVSQEDPEVQFNWYVDGVEVHNAKTKPREEQFNSTYRVVSVLTVLHQDWLNGKEYKCKVSNKGLPSSIEKTISKAKGQPREPQVYTLPPSQEEMTKNQVSLTCLVKGFYPSDIAVEWESNGQPENNYKTTPPVLDSDGSFFLYSRLTVDKSRWQEGNVFSCSVMHEALHNHYTQKSLSLSLGK

SEQ ID NO: 552 - DNA, 2118 bp, synthetic construct
  misc_feature 1..2118: note = Synthetic
  source 1..2118: mol_type = other DNA
gaggtgcagctggtgcagagcggagcagaggtgaagaagccaggggccagcgtgaaggtgagctgtaaggctagtgggtacacatttacaaactattggctgggatggattaagcaggccccaggccaaggactggagtggataggagacatataccccggaggagactatatcgtgtacaacgagaagttcaagggcaaggccacactcaccgctgatacaagcatcagcaccgcctacatggagctgagccgactgagaagcgacgacacagcagtgtattactgcgccagacccaacctgcccaaggaccactggggacaaggcaccaccgtgaccgtgtcttccgctagcaccaagggcccctccgtgttccctctggccccatgctcccggtccacctccgagtccaccgccgctctgggctgtctggtgaaggactacttccctgagcccgtgaccgtgagctggaactctggcgccctgacctccggcgtgcacaccttccctgccgtgctgcagtcctccggcctgtactccctgtcctccgtggtgaccgtgccttcctcctccctgggcaccaagacctacacctgcaacgtggaccacaagccttccaacaccaaggtggacaagcgggtggagtccaagtacggccctccttgccctccctgccctgcccctgagttcctgggcggaccctccgtgttcctgttccctcctaagcctaaggacaccctgatgatctcccggacccctgaggtgacctgcgtggtggtggacgtgtcccaggaagatcctgaggtccagttcaattggtacgtggatggcgtggaggtgcacaacgccaagaccaagcctcgggaggaacagttcaactccacctaccgggtggtgtctgtgctgaccgtgctgcaccaggactggctgaacggcaaggaatacaagtgcaaggtcagcaacaagggcctgccctcctccatcgagaaaaccatctccaaggccaagggccagcctcgcgagcctcaggtgtacaccctgcctcctagccaggaagagatgaccaagaatcaggtgtccctgacatgcctggtgaagggcttctacccttccgatatcgccgtggagtgggagagcaacggccagccagagaacaactacaagaccacccctcctgtgctggactccgacggctccttcttcctgtactccaggctgaccgtggacaagtcccggtggcaggaaggcaacgtcttttcctgctccgtgatgcacgaggccctgcacaaccactacacccagaagtccctgtccctgtctctgggcaagggtggaggtgggtctgggggtggcgggtcaggtggaggaggttcagacatccagatgacccagagccctagcagcctgagcgctagcgtgggcgacagggtgaccatcacctgcaaggccagccaggatgtgacccctgccgtggcctggtaccagcagaagcccggcaaggcccccaagctgctgatctacagcaccagcagcaggtacaccggcgtgcccagcaggtttagcggaagcggcagcggcaccgacttcaccttcaccatcagcagcctgcagcccgaggacatcgccacctactactgccagcagcactacaccacccctctgaccttcggctgtggcaccaagctggagatcaagagaggtggaggcggctcaggggggggtggatcagggggaggaggatcagggggaggcggtagtgaggtgcagctggtggagagcggaggaggactggtgcaacccggaggcagcctgagactgagctgcgctgccagcggcttcaccttcagcagctacgacatgagctgggtgagacaggcccctggcaaatgtctggagtgggtggccaccatctccgatgcgggcggctacatctattactccgacagcgtgaagggcaggttcaccatcagcagggacaacgccaagaacagcctgtacctgcagatgaacagcctgagggatgaggacaccgccgtgtacatctgcgccagggagttcggcaaaaggtacgccctggactactggggccagggcacaaccgtgaccgtgagcagctga

SEQ ID NO: 553 - protein, 219 aa, synthetic construct
  REGION 1..219: note = Synthetic
DIVMTQSPLSLPVTPGEPASISCRSSKSLLHSQGITYLYWYLQKPGQSPQLLIYQVSNLASGVPDRFSGSGSGTDFTLKISRVEAEDVGVYYCAQYLELPWTFGGGTKVEIKRTVAAPSVFIFPPSDEQLKSGTASVVCLLNNFYPREAKVQWKVDNALQSGNSQESVTEQDSKDSTYSLSSTLTLSKADYEKHKVYACEVTHQGLSSPVTKSFNRGEC

SEQ ID NO: 554 - DNA, 660 bp, synthetic construct
  misc_feature 1..660: note = Synthetic
  source 1..660: mol_type = other DNA
gacattgtgatgacccagagccccctgagcctccccgtgacccctggagaacccgccagcataagctgcagatcctccaaaagcctgctgcactcccagggaataacctacctgtattggtacctgcagaaacccggccaatccccccaactcctgatataccaagtgtccaacctggcctccggcgtgcccgacagattctccggctccggcagcggtaccgacttcaccctcaaaatctccagagtggaagcagaagacgtcggcgtgtactactgcgcccagtacctggaactgccctggaccttcggcggcggcaccaaggtggaaatcaagagaaccgtggccgctccctccgtgttcatcttcccaccatctgacgagcagctgaagtccggcaccgcttctgtcgtgtgcctgctgaacaacttctaccctcgggaagccaaggtgcagtggaaggtggacaatgccctgcagtccggcaactcccaagagtctgtgaccgagcaggactccaaggacagcacctactccctgtcctctaccctgaccctgtccaaggccgactacgagaagcacaaggtgtacgcctgcgaagtgacccaccagggactgtctagccccgtgaccaagtccttcaacagaggcgagtgctga

SEQ ID NO: 555 - DNA, 2118 bp, synthetic construct
  misc_feature 1..2118: note = Synthetic
  source 1..2118: mol_type = other DNA
gaggtgcagctggtgcagagcggagcagaggtgaagaagccaggggccagcgtgaaggtgagctgtaaggctagtgggtacacatttacaaactattggctgggatggattaagcaggccccaggccaaggactggagtggataggagacatataccccggaggagactatatcgtgtacaacgagaagttcaagggcaaggccacactcaccgctgatacaagcatcagcaccgcctacatggagctgagccgactgagaagcgacgacacagcagtgtattactgcgccagacccaacctgcccaaggaccactggggacaaggcaccaccgtgaccgtgtcttccgctagcaccaagggcccctccgtgttccctctggccccatgctcccggtccacctccgagtccaccgccgctctgggctgtctggtgaaggactacttccctgagcccgtgaccgtgagctggaactctggcgccctgacctccggcgtgcacaccttccctgccgtgctgcagtcctccggcctgtactccctgtcctccgtggtgaccgtgccttcctcctccctgggcaccaagacctacacctgcaacgtggaccacaagccttccaacaccaaggtggacaagcgggtggagtccaagtacggccctccttgccctccctgccctgcccctgagttcctgggcggaccctccgtgttcctgttccctcctaagcctaaggacaccctgatgatctcccggacccctgaggtgacctgcgtggtggtggacgtgtcccaggaagatcctgaggtccagttcaattggtacgtggatggcgtggaggtgcacaacgccaagaccaagcctcgggaggaacagttcaactccacctaccgggtggtgtctgtgctgaccgtgctgcaccaggactggctgaacggcaaggaatacaagtgcaaggtcagcaacaagggcctgccctcctccatcgagaaaaccatctccaaggccaagggccagcctcgcgagcctcaggtgtacaccctgcctcctagccaggaagagatgaccaagaatcaggtgtccctgacatgcctggtgaagggcttctacccttccgatatcgccgtggaatgggagagcaatggccagcctgagaacaactacaagacaacccctcctgtgctggactccgacggctccttctttctgtactctcgcctgaccgtggacaagtccagatggcaagagggcaacgtgttctcctgctccgtgatgcacgaggccctgcacaatcactacacccagaagtccctgtctctgtccctcggaaaaggcggcggaggatctggcggaggcggtagcggtggtggcggatctgatattcagatgacccagtctccttccagcctgtccgcttctgtgggcgacagagtgaccatcacatgcaaggccagccaggatgtgacccctgctgtggcttggtatcagcagaagcctggcaaggcccctaagctgctgatctactccacctcctccagatacacaggcgtgccctccagattctccggctctggctctggcaccgactttacctttacaatctccagcctgcagcctgaggacattgccacctactactgccagcagcactacaccacacctctgacctttggctgcggcaccaagctggaaatcaagagaggtggcggaggaagcggaggcggcggttcaggtggcggtggttcaggcggtggtggatctgaagttcagctggtggaatctggcggcggattggttcaaccaggcggctctctgagactgtcttgtgccgcttccggcttcaccttctccagctacgacatgtcctgggtccgacaggcccctggaaagtgtctggaatgggtcgccaccatctctgacgctggcggctacatctactaccgggactctgtgaagggcagattcaccatcagccgggacaatgccaagaactccctgtacctgcagatgaacagtctgcgcgacgaggacaccgccgtgtacatctgtgctagagagctgccttggcgctacgccctggattattggggccagggcacaacagtgacagtgtcctcttga